European Patent Application EP 4 166 158 A1, published April 19, 2023. Title: Nucleic acid lipid particle vaccine in which SARA-CoV-2 mRNA is encapusulated. Applicant: DAIICHI SANKYO COMPANY, LIMITED The University of Tokyo. The sequence listing filed with the application follows.

SEQUENCE LISTING (107 sequences)

SEQ ID NO: 1 - DNA, 4042 bp, Artificial Sequence
  DNA insert
gtaatacgactcactataaggagacccaagctacatttgcttctgacacaactgtgttcactagcaacctcaaacagacaccgccaccatgtttgtttttcttgttttattgccactagtctctagtcagtgtgttaatcttacaaccagaactcaattaccccctgcatacactaattctttcacacgtggtgtttattaccctgacaaagttttcagatcctcagttttacattcaactcaggacttgttcttacctttcttttccaatgttacttggttccatgctatacatgtctctgggaccaatggtactaagaggtttgataaccctgtcctaccatttaatgatggtgtttattttgcttccactgagaagtctaacataataagaggctggatttttggtactactttagattcgaagacccagtccctacttattgttaataacgctactaatgttgttattaaagtctgtgaatttcaattttgtaatgatccatttttgggtgtttattaccacaaaaacaacaaaagttggatggaaagtgagttcagagtttattctagtgcgaataattgcacttttgaatatgtctctcagccttttcttatggaccttgaaggaaaacagggtaatttcaaaaatcttagggaatttgtgtttaagaatattgatggttattttaaaatatattctaagcacacgcctattaatttagtgcgtgatctccctcagggtttttcggctttagaaccattggtagatttgccaataggtattaacatcactaggtttcaaactttacttgctttacatagaagttatttgactcctggtgattcttcttcaggttggacagctggtgctgcagcttattatgtgggttatcttcaacctaggacttttctattaaaatataatgaaaatggaaccattacagatgctgtagactgtgcacttgaccctctctcagaaacaaagtgtacgttgaaatccttcactgtagaaaaaggaatctatcaaacttctaactttagagtccaaccaacagaatctattgttagatttcctaatattacaaacttgtgcccttttggtgaagtttttaacgccaccagatttgcatctgtttatgcttggaacaggaagagaatcagcaactgtgttgctgattattctgtcctatataattccgcatcattttccacttttaagtgttatggagtgtctcctactaaattaaatgatctctgctttactaatgtctatgcagattcatttgtaattagaggtgatgaagtcagacaaatcgctccagggcaaactggaaagattgctgattataattataaattaccagatgattttacaggctgcgttatagcttggaattctaacaatcttgattctaaggttggtggtaattataattacctgtatagattgtttaggaagtctaatctcaaaccttttgagagagatatttcaactgaaatctatcaggccggtagcacaccttgtaatggtgttgaaggttttaattgttactttcctttacaatcatatggtttccaacccactaatggtgttggttaccaaccatacagagtagtagtactttcttttgaacttctacatgcaccagcaactgtttgtggacctaaaaagtctactaatttggttaaaaacaaatgtgtcaatttcaacttcaatggtttaacaggcacaggtgttcttactgagtctaacaaaaagtttctgcctttccaacaatttggcagagacattgctgacactactgatgctgtccgtgatccacagacacttgagattcttgacattacaccatgttcttttggtggtgtcagtgttataacaccaggaacaaatacttctaaccaggttgctgttctttatcaggatgttaactgcacagaagtccctgttgctattcatgcagatcaacttactcctacttggcgtgtttattctacaggttctaatgtttttcaaacacgtgcaggctgtttaataggggctgaacatgtcaacaactcatatgagtgtgacatacccattggtgcaggtatatgcgctagttatcagactcagactaattctcctcggcgggcacgtagtgtagctagtcaatccatcattgcctacactatgtcacttggtgcagaaaattcagttgcttactctaataactctattgccatacccacaaattttactattagtgttaccacagaaattctaccagtgtctatgaccaagacatcagtagattgtacaatgtacatttgtggtgattcaactgaatgcagcaatcttttgttgcaatatggcagtttttgtacacaattaaaccgtgctttaactggaatagctgttgaacaagacaaaaacacccaagaagtttttgcacaagtcaaacaaatttacaaaacaccaccaattaaagattttggtggttttaatttttcacaaatattaccagatccatcaaaaccaagcaagaggtcatttattgaagatctacttttcaacaaagtgacacttgcagatgctggcttcatcaaacaatatggtgattgccttggtgatattgctgctagagacctcatttgtgcacaaaagtttaacggccttactgttttgccacctttgctcacagatgaaatgattgctcaatacacttctgcactgttagcgggtacaatcacttctggttggacctttggtgcaggtgctgcattacaaataccatttgctatgcaaatggcttataggtttaatggtattggagttacacagaatgttctctatgagaaccaaaaattgattgccaaccaatttaatagtgctattggcaaaattcaagactcactttcttccacagcaagtgcacttggaaaacttcaagatgtggtcaaccaaaatgcacaagctttaaacacgcttgttaaacaacttagctccaattttggtgcaatttcaagtgttttaaatgatatcctttcacgtcttgacaaagttgaggctgaagtgcaaattgataggttgatcacaggcagacttcaaagtttgcagacatatgtgactcaacaattaattagagctgcagaaatcagagcttctgctaatcttgctgctactaaaatgtcagagtgtgtacttggacaatcaaaaagagttgatttttgtggaaagggctatcatcttatgtccttccctcagtcagcacctcatggtgtagtcttcttgcatgtgacttatgtccctgcacaagaaaagaacttcacaactgctcctgccatttgtcatgatggaaaagcacactttcctcgtgaaggtgtctttgtttcaaatggcacacactggtttgtaacacaaaggaatttttatgaaccacaaatcattactacagacaacacatttgtgtctggtaactgtgatgttgtaataggaattgtcaacaacacagtttatgatcctttgcaacctgaattagactcattcaaggaggagttagataaatattttaagaatcatacatcaccagatgttgatttaggtgacatctctggcattaatgcttcagttgtaaacattcaaaaagaaattgaccgcctcaatgaggttgccaagaatttaaatgaatctctcatcgatctccaagaacttggaaagtatgagcagtatataaaatggccatggtacatttggctaggttttatagctggcttgattgccatagtaatggtgacaattatgctttgctgtatgaccagttgctgtagttgtctcaagggctgttgttcttgtggatcctgctgcaaatttgatgaagacgactctgagccagtgctcaaaggagtcaaattacattacacatgagctcgctttcttgctgtccaatttctattaaaggttcctttgttccctaagtccaactactaaactgggggatattatgaagggccttgagcatctggattctgcctaataaaaaacatttattttcattgc

SEQ ID NO: 2 - DNA, 19 bp, Artificial Sequence
  primer
gtaatacgactcactataa

SEQ ID NO: 3 - DNA, 129 bp, Artificial Sequence
  primer
ttttttttttttttttttttttttttttttttttttttttttttttttttttttttttttttttttttttttttttttttttttttttttttttttttttgcaatgaaaataaatgttttttattaggc

SEQ ID NO: 4 - DNA, 4142 bp, Artificial Sequence
  template DNA
gtaatacgactcactataaggagacccaagctacatttgcttctgacacaactgtgttcactagcaacctcaaacagacaccgccaccatgtttgtttttcttgttttattgccactagtctctagtcagtgtgttaatcttacaaccagaactcaattaccccctgcatacactaattctttcacacgtggtgtttattaccctgacaaagttttcagatcctcagttttacattcaactcaggacttgttcttacctttcttttccaatgttacttggttccatgctatacatgtctctgggaccaatggtactaagaggtttgataaccctgtcctaccatttaatgatggtgtttattttgcttccactgagaagtctaacataataagaggctggatttttggtactactttagattcgaagacccagtccctacttattgttaataacgctactaatgttgttattaaagtctgtgaatttcaattttgtaatgatccatttttgggtgtttattaccacaaaaacaacaaaagttggatggaaagtgagttcagagtttattctagtgcgaataattgcacttttgaatatgtctctcagccttttcttatggaccttgaaggaaaacagggtaatttcaaaaatcttagggaatttgtgtttaagaatattgatggttattttaaaatatattctaagcacacgcctattaatttagtgcgtgatctccctcagggtttttcggctttagaaccattggtagatttgccaataggtattaacatcactaggtttcaaactttacttgctttacatagaagttatttgactcctggtgattcttcttcaggttggacagctggtgctgcagcttattatgtgggttatcttcaacctaggacttttctattaaaatataatgaaaatggaaccattacagatgctgtagactgtgcacttgaccctctctcagaaacaaagtgtacgttgaaatccttcactgtagaaaaaggaatctatcaaacttctaactttagagtccaaccaacagaatctattgttagatttcctaatattacaaacttgtgcccttttggtgaagtttttaacgccaccagatttgcatctgtttatgcttggaacaggaagagaatcagcaactgtgttgctgattattctgtcctatataattccgcatcattttccacttttaagtgttatggagtgtctcctactaaattaaatgatctctgctttactaatgtctatgcagattcatttgtaattagaggtgatgaagtcagacaaatcgctccagggcaaactggaaagattgctgattataattataaattaccagatgattttacaggctgcgttatagcttggaattctaacaatcttgattctaaggttggtggtaattataattacctgtatagattgtttaggaagtctaatctcaaaccttttgagagagatatttcaactgaaatctatcaggccggtagcacaccttgtaatggtgttgaaggttttaattgttactttcctttacaatcatatggtttccaacccactaatggtgttggttaccaaccatacagagtagtagtactttcttttgaacttctacatgcaccagcaactgtttgtggacctaaaaagtctactaatttggttaaaaacaaatgtgtcaatttcaacttcaatggtttaacaggcacaggtgttcttactgagtctaacaaaaagtttctgcctttccaacaatttggcagagacattgctgacactactgatgctgtccgtgatccacagacacttgagattcttgacattacaccatgttcttttggtggtgtcagtgttataacaccaggaacaaatacttctaaccaggttgctgttctttatcaggatgttaactgcacagaagtccctgttgctattcatgcagatcaacttactcctacttggcgtgtttattctacaggttctaatgtttttcaaacacgtgcaggctgtttaataggggctgaacatgtcaacaactcatatgagtgtgacatacccattggtgcaggtatatgcgctagttatcagactcagactaattctcctcggcgggcacgtagtgtagctagtcaatccatcattgcctacactatgtcacttggtgcagaaaattcagttgcttactctaataactctattgccatacccacaaattttactattagtgttaccacagaaattctaccagtgtctatgaccaagacatcagtagattgtacaatgtacatttgtggtgattcaactgaatgcagcaatcttttgttgcaatatggcagtttttgtacacaattaaaccgtgctttaactggaatagctgttgaacaagacaaaaacacccaagaagtttttgcacaagtcaaacaaatttacaaaacaccaccaattaaagattttggtggttttaatttttcacaaatattaccagatccatcaaaaccaagcaagaggtcatttattgaagatctacttttcaacaaagtgacacttgcagatgctggcttcatcaaacaatatggtgattgccttggtgatattgctgctagagacctcatttgtgcacaaaagtttaacggccttactgttttgccacctttgctcacagatgaaatgattgctcaatacacttctgcactgttagcgggtacaatcacttctggttggacctttggtgcaggtgctgcattacaaataccatttgctatgcaaatggcttataggtttaatggtattggagttacacagaatgttctctatgagaaccaaaaattgattgccaaccaatttaatagtgctattggcaaaattcaagactcactttcttccacagcaagtgcacttggaaaacttcaagatgtggtcaaccaaaatgcacaagctttaaacacgcttgttaaacaacttagctccaattttggtgcaatttcaagtgttttaaatgatatcctttcacgtcttgacaaagttgaggctgaagtgcaaattgataggttgatcacaggcagacttcaaagtttgcagacatatgtgactcaacaattaattagagctgcagaaatcagagcttctgctaatcttgctgctactaaaatgtcagagtgtgtacttggacaatcaaaaagagttgatttttgtggaaagggctatcatcttatgtccttccctcagtcagcacctcatggtgtagtcttcttgcatgtgacttatgtccctgcacaagaaaagaacttcacaactgctcctgccatttgtcatgatggaaaagcacactttcctcgtgaaggtgtctttgtttcaaatggcacacactggtttgtaacacaaaggaatttttatgaaccacaaatcattactacagacaacacatttgtgtctggtaactgtgatgttgtaataggaattgtcaacaacacagtttatgatcctttgcaacctgaattagactcattcaaggaggagttagataaatattttaagaatcatacatcaccagatgttgatttaggtgacatctctggcattaatgcttcagttgtaaacattcaaaaagaaattgaccgcctcaatgaggttgccaagaatttaaatgaatctctcatcgatctccaagaacttggaaagtatgagcagtatataaaatggccatggtacatttggctaggttttatagctggcttgattgccatagtaatggtgacaattatgctttgctgtatgaccagttgctgtagttgtctcaagggctgttgttcttgtggatcctgctgcaaatttgatgaagacgactctgagccagtgctcaaaggagtcaaattacattacacatgagctcgctttcttgctgtccaatttctattaaaggttcctttgttccctaagtccaactactaaactgggggatattatgaagggccttgagcatctggattctgcctaataaaaaacatttattttcattgcaaaaaaaaaaaaaaaaaaaaaaaaaaaaaaaaaaaaaaaaaaaaaaaaaaaaaaaaaaaaaaaaaaaaaaaaaaaaaaaaaaaaaaaaaaaaaaaaaaaa

SEQ ID NO: 5 - RNA, 4142 nt, Artificial Sequence
  SARS-Cov-2 S full mRNA-001
guaauacgacucacuauaaggagacccaagcuacauuugcuucugacacaacuguguucacuagcaaccucaaacagacaccgccaccauguuuguuuuucuuguuuuauugccacuagucucuagucaguguguuaaucuuacaaccagaacucaauuacccccugcauacacuaauucuuucacacgugguguuuauuacccugacaaaguuuucagauccucaguuuuacauucaacucaggacuuguucuuaccuuucuuuuccaauguuacuugguuccaugcuauacaugucucugggaccaaugguacuaagagguuugauaacccuguccuaccauuuaaugaugguguuuauuuugcuuccacugagaagucuaacauaauaagaggcuggauuuuugguacuacuuuagauucgaagacccagucccuacuuauuguuaauaacgcuacuaauguuguuauuaaagucugugaauuucaauuuuguaaugauccauuuuuggguguuuauuaccacaaaaacaacaaaaguuggauggaaagugaguucagaguuuauucuagugcgaauaauugcacuuuugaauaugucucucagccuuuucuuauggaccuugaaggaaaacaggguaauuucaaaaaucuuagggaauuuguguuuaagaauauugaugguuauuuuaaaauauauucuaagcacacgccuauuaauuuagugcgugaucucccucaggguuuuucggcuuuagaaccauugguagauuugccaauagguauuaacaucacuagguuucaaacuuuacuugcuuuacauagaaguuauuugacuccuggugauucuucuucagguuggacagcuggugcugcagcuuauuauguggguuaucuucaaccuaggacuuuucuauuaaaauauaaugaaaauggaaccauuacagaugcuguagacugugcacuugacccucucucagaaacaaaguguacguugaaauccuucacuguagaaaaaggaaucuaucaaacuucuaacuuuagaguccaaccaacagaaucuauuguuagauuuccuaauauuacaaacuugugcccuuuuggugaaguuuuuaacgccaccagauuugcaucuguuuaugcuuggaacaggaagagaaucagcaacuguguugcugauuauucuguccuauauaauuccgcaucauuuuccacuuuuaaguguuauggagugucuccuacuaaauuaaaugaucucugcuuuacuaaugucuaugcagauucauuuguaauuagaggugaugaagucagacaaaucgcuccagggcaaacuggaaagauugcugauuauaauuauaaauuaccagaugauuuuacaggcugcguuauagcuuggaauucuaacaaucuugauucuaagguuggugguaauuauaauuaccuguauagauuguuuaggaagucuaaucucaaaccuuuugagagagauauuucaacugaaaucuaucaggccgguagcacaccuuguaaugguguugaagguuuuaauuguuacuuuccuuuacaaucauaugguuuccaacccacuaaugguguugguuaccaaccauacagaguaguaguacuuucuuuugaacuucuacaugcaccagcaacuguuuguggaccuaaaaagucuacuaauuugguuaaaaacaaaugugucaauuucaacuucaaugguuuaacaggcacagguguucuuacugagucuaacaaaaaguuucugccuuuccaacaauuuggcagagacauugcugacacuacugaugcuguccgugauccacagacacuugagauucuugacauuacaccauguucuuuugguggugucaguguuauaacaccaggaacaaauacuucuaaccagguugcuguucuuuaucaggauguuaacugcacagaagucccuguugcuauucaugcagaucaacuuacuccuacuuggcguguuuauucuacagguucuaauguuuuucaaacacgugcaggcuguuuaauaggggcugaacaugucaacaacucauaugagugugacauacccauuggugcagguauaugcgcuaguuaucagacucagacuaauucuccucggcgggcacguaguguagcuagucaauccaucauugccuacacuaugucacuuggugcagaaaauucaguugcuuacucuaauaacucuauugccauacccacaaauuuuacuauuaguguuaccacagaaauucuaccagugucuaugaccaagacaucaguagauuguacaauguacauuuguggugauucaacugaaugcagcaaucuuuuguugcaauauggcaguuuuuguacacaauuaaaccgugcuuuaacuggaauagcuguugaacaagacaaaaacacccaagaaguuuuugcacaagucaaacaaauuuacaaaacaccaccaauuaaagauuuuggugguuuuaauuuuucacaaauauuaccagauccaucaaaaccaagcaagaggucauuuauugaagaucuacuuuucaacaaagugacacuugcagaugcuggcuucaucaaacaauauggugauugccuuggugauauugcugcuagagaccucauuugugcacaaaaguuuaacggccuuacuguuuugccaccuuugcucacagaugaaaugauugcucaauacacuucugcacuguuagcggguacaaucacuucugguuggaccuuuggugcaggugcugcauuacaaauaccauuugcuaugcaaauggcuuauagguuuaaugguauuggaguuacacagaauguucucuaugagaaccaaaaauugauugccaaccaauuuaauagugcuauuggcaaaauucaagacucacuuucuuccacagcaagugcacuuggaaaacuucaagauguggucaaccaaaaugcacaagcuuuaaacacgcuuguuaaacaacuuagcuccaauuuuggugcaauuucaaguguuuuaaaugauauccuuucacgucuugacaaaguugaggcugaagugcaaauugauagguugaucacaggcagacuucaaaguuugcagacauaugugacucaacaauuaauuagagcugcagaaaucagagcuucugcuaaucuugcugcuacuaaaaugucagaguguguacuuggacaaucaaaaagaguugauuuuuguggaaagggcuaucaucuuauguccuucccucagucagcaccucaugguguagucuucuugcaugugacuuaugucccugcacaagaaaagaacuucacaacugcuccugccauuugucaugauggaaaagcacacuuuccucgugaaggugucuuuguuucaaauggcacacacugguuuguaacacaaaggaauuuuuaugaaccacaaaucauuacuacagacaacacauuugugucugguaacugugauguuguaauaggaauugucaacaacacaguuuaugauccuuugcaaccugaauuagacucauucaaggaggaguuagauaaauauuuuaagaaucauacaucaccagauguugauuuaggugacaucucuggcauuaaugcuucaguuguaaacauucaaaaagaaauugaccgccucaaugagguugccaagaauuuaaaugaaucucucaucgaucuccaagaacuuggaaaguaugagcaguauauaaaauggccaugguacauuuggcuagguuuuauagcuggcuugauugccauaguaauggugacaauuaugcuuugcuguaugaccaguugcuguaguugucucaagggcuguuguucuuguggauccugcugcaaauuugaugaagacgacucugagccagugcucaaaggagucaaauuacauuacacaugagcucgcuuucuugcuguccaauuucuauuaaagguuccuuuguucccuaaguccaacuacuaaacugggggauauuaugaagggccuugagcaucuggauucugccuaauaaaaaacauuuauuuucauugcaaaaaaaaaaaaaaaaaaaaaaaaaaaaaaaaaaaaaaaaaaaaaaaaaaaaaaaaaaaaaaaaaaaaaaaaaaaaaaaaaaaaaaaaaaaaaaaaaaaa

SEQ ID NO: 6 - protein, 1273 aa, severe acute respiratory syndrome coronavirus 2
MFVFLVLLPLVSSQCVNLTTRTQLPPAYTNSFTRGVYYPDKVFRSSVLHSTQDLFLPFFSNVTWFHAIHVSGTNGTKRFDNPVLPFNDGVYFASTEKSNIIRGWIFGTTLDSKTQSLLIVNNATNVVIKVCEFQFCNDPFLGVYYHKNNKSWMESEFRVYSSANNCTFEYVSQPFLMDLEGKQGNFKNLREFVFKNIDGYFKIYSKHTPINLVRDLPQGFSALEPLVDLPIGINITRFQTLLALHRSYLTPGDSSSGWTAGAAAYYVGYLQPRTFLLKYNENGTITDAVDCALDPLSETKCTLKSFTVEKGIYQTSNFRVQPTESIVRFPNITNLCPFGEVFNATRFASVYAWNRKRISNCVADYSVLYNSASFSTFKCYGVSPTKLNDLCFTNVYADSFVIRGDEVRQIAPGQTGKIADYNYKLPDDFTGCVIAWNSNNLDSKVGGNYNYLYRLFRKSNLKPFERDISTEIYQAGSTPCNGVEGFNCYFPLQSYGFQPTNGVGYQPYRVVVLSFELLHAPATVCGPKKSTNLVKNKCVNFNFNGLTGTGVLTESNKKFLPFQQFGRDIADTTDAVRDPQTLEILDITPCSFGGVSVITPGTNTSNQVAVLYQDVNCTEVPVAIHADQLTPTWRVYSTGSNVFQTRAGCLIGAEHVNNSYECDIPIGAGICASYQTQTNSPRRARSVASQSIIAYTMSLGAENSVAYSNNSIAIPTNFTISVTTEILPVSMTKTSVDCTMYICGDSTECSNLLLQYGSFCTQLNRALTGIAVEQDKNTQEVFAQVKQIYKTPPIKDFGGFNFSQILPDPSKPSKRSFIEDLLFNKVTLADAGFIKQYGDCLGDIAARDLICAQKFNGLTVLPPLLTDEMIAQYTSALLAGTITSGWTFGAGAALQIPFAMQMAYRFNGIGVTQNVLYENQKLIANQFNSAIGKIQDSLSSTASALGKLQDVVNQNAQALNTLVKQLSSNFGAISSVLNDILSRLDKVEAEVQIDRLITGRLQSLQTYVTQQLIRAAEIRASANLAATKMSECVLGQSKRVDFCGKGYHLMSFPQSAPHGVVFLHVTYVPAQEKNFTTAPAICHDGKAHFPREGVFVSNGTHWFVTQRNFYEPQIITTDNTFVSGNCDVVIGIVNNTVYDPLQPELDSFKEELDKYFKNHTSPDVDLGDISGINASVVNIQKEIDRLNEVAKNLNESLIDLQELGKYEQYIKWPWYIWLGFIAGLIAIVMVTIMLCCMTSCCSCLKGCCSCGSCCKFDEDDSEPVLKGVKLHYT

SEQ ID NO: 7 - DNA, 931 bp, Artificial Sequence
  DNA insert
gtaatacgactcactataaggagacccaagctacatttgcttctgacacaactgtgttcactagcaacctcaaacagacaccgccaccatgtttgtttttcttgttttattgccactagtctctagtagagtccaaccaacagaatctattgttagatttcctaatattacaaacttgtgcccttttggtgaagtttttaacgccaccagatttgcatctgtttatgcttggaacaggaagagaatcagcaactgtgttgctgattattctgtcctatataattccgcatcattttccacttttaagtgttatggagtgtctcctactaaattaaatgatctctgctttactaatgtctatgcagattcatttgtaattagaggtgatgaagtcagacaaatcgctccagggcaaactggaaagattgctgattataattataaattaccagatgattttacaggctgcgttatagcttggaattctaacaatcttgattctaaggttggtggtaattataattacctgtatagattgtttaggaagtctaatctcaaaccttttgagagagatatttcaactgaaatctatcaggccggtagcacaccttgtaatggtgttgaaggttttaattgttactttcctttacaatcatatggtttccaacccactaatggtgttggttaccaaccatacagagtagtagtactttcttttgaacttctacatgcaccagcaactgtttgtggacctaaaaagtctactaatttggttaaaaacaaatgtgtcaatttctgagctcgctttcttgctgtccaatttctattaaaggttcctttgttccctaagtccaactactaaactgggggatattatgaagggccttgagcatctggattctgcctaataaaaaacatttattttcattgc

SEQ ID NO: 8 - DNA, 1031 bp, Artificial Sequence
  template DNA
gtaatacgactcactataaggagacccaagctacatttgcttctgacacaactgtgttcactagcaacctcaaacagacaccgccaccatgtttgtttttcttgttttattgccactagtctctagtagagtccaaccaacagaatctattgttagatttcctaatattacaaacttgtgcccttttggtgaagtttttaacgccaccagatttgcatctgtttatgcttggaacaggaagagaatcagcaactgtgttgctgattattctgtcctatataattccgcatcattttccacttttaagtgttatggagtgtctcctactaaattaaatgatctctgctttactaatgtctatgcagattcatttgtaattagaggtgatgaagtcagacaaatcgctccagggcaaactggaaagattgctgattataattataaattaccagatgattttacaggctgcgttatagcttggaattctaacaatcttgattctaaggttggtggtaattataattacctgtatagattgtttaggaagtctaatctcaaaccttttgagagagatatttcaactgaaatctatcaggccggtagcacaccttgtaatggtgttgaaggttttaattgttactttcctttacaatcatatggtttccaacccactaatggtgttggttaccaaccatacagagtagtagtactttcttttgaacttctacatgcaccagcaactgtttgtggacctaaaaagtctactaatttggttaaaaacaaatgtgtcaatttctgagctcgctttcttgctgtccaatttctattaaaggttcctttgttccctaagtccaactactaaactgggggatattatgaagggccttgagcatctggattctgcctaataaaaaacatttattttcattgcaaaaaaaaaaaaaaaaaaaaaaaaaaaaaaaaaaaaaaaaaaaaaaaaaaaaaaaaaaaaaaaaaaaaaaaaaaaaaaaaaaaaaaaaaaaaaaaaaaaa

SEQ ID NO: 9 - RNA, 1013 nt, Artificial Sequence
  SARS-CoV-2 RBD mRNA-002
aggagacccaagcuacauuugcuucugacacaacuguguucacuagcaaccucaaacagacaccgccaccauguuuguuuuucuuguuuuauugccacuagucucuaguagaguccaaccaacagaaucuauuguuagauuuccuaauauuacaaacuugugcccuuuuggugaaguuuuuaacgccaccagauuugcaucuguuuaugcuuggaacaggaagagaaucagcaacuguguugcugauuauucuguccuauauaauuccgcaucauuuuccacuuuuaaguguuauggagugucuccuacuaaauuaaaugaucucugcuuuacuaaugucuaugcagauucauuuguaauuagaggugaugaagucagacaaaucgcuccagggcaaacuggaaagauugcugauuauaauuauaaauuaccagaugauuuuacaggcugcguuauagcuuggaauucuaacaaucuugauucuaagguuggugguaauuauaauuaccuguauagauuguuuaggaagucuaaucucaaaccuuuugagagagauauuucaacugaaaucuaucaggccgguagcacaccuuguaaugguguugaagguuuuaauuguuacuuuccuuuacaaucauaugguuuccaacccacuaaugguguugguuaccaaccauacagaguaguaguacuuucuuuugaacuucuacaugcaccagcaacuguuuguggaccuaaaaagucuacuaauuugguuaaaaacaaaugugucaauuucugagcucgcuuucuugcuguccaauuucuauuaaagguuccuuuguucccuaaguccaacuacuaaacugggggauauuaugaagggccuugagcaucuggauucugccuaauaaaaaacauuuauuuucauugcaaaaaaaaaaaaaaaaaaaaaaaaaaaaaaaaaaaaaaaaaaaaaaaaaaaaaaaaaaaaaaaaaaaaaaaaaaaaaaaaaaaaaaaaaaaaaaaaaaaa

SEQ ID NO: 10 - protein, 236 aa, Artificial Sequence
  spike protein signal sequence added SARS-CoV-2 RBD
MFVFLVLLPLVSSRVQPTESIVRFPNITNLCPFGEVFNATRFASVYAWNRKRISNCVADYSVLYNSASFSTFKCYGVSPTKLNDLCFTNVYADSFVIRGDEVRQIAPGQTGKIADYNYKLPDDFTGCVIAWNSNNLDSKVGGNYNYLYRLFRKSNLKPFERDISTEIYQAGSTPCNGVEGFNCYFPLQSYGFQPTNGVGYQPYRVVVLSFELLHAPATVCGPKKSTNLVKNKCVNF

SEQ ID NO: 11 - protein, 223 aa, severe acute respiratory syndrome coronavirus 2
RVQPTESIVRFPNITNLCPFGEVFNATRFASVYAWNRKRISNCVADYSVLYNSASFSTFKCYGVSPTKLNDLCFTNVYADSFVIRGDEVRQIAPGQTGKIADYNYKLPDDFTGCVIAWNSNNLDSKVGGNYNYLYRLFRKSNLKPFERDISTEIYQAGSTPCNGVEGFNCYFPLQSYGFQPTNGVGYQPYRVVVLSFELLHAPATVCGPKKSTNLVKNKCVNF

SEQ ID NO: 12 - DNA, 4054 bp, Artificial Sequence
  DNA insert
gctagcgtaatacgactcactataaggagacccaagctacatttgcttctgacacaactgtgttcactagcaacctcaaacagacaccgccaccatgttcgtgttcctggtgctgctgcccctggtgagcagccagtgcgtgaacctgaccaccagaacacagctgcccccagcctacaccaacagcttcaccagaggcgtgtactaccccgacaaggtgttcagaagcagcgtgctgcacagcacccaggacctgttcctgcccttcttcagcaacgtgacctggttccacgccatccacgtgagcggcaccaacggcaccaagagattcgacaaccccgtgctgcccttcaacgacggggtgtacttcgccagcaccgagaagtccaacatcatcagaggctggatcttcggcaccacactggacagcaagacccagagcctgctgatcgtgaacaacgccaccaacgtggtcatcaaagtgtgcgagttccagttctgcaacgaccccttcctgggcgtctactaccacaagaacaacaagagctggatggaaagcgagttccgggtgtacagcagcgccaacaactgcaccttcgagtacgtgagccagcccttcctgatggacctggaaggcaagcagggcaacttcaagaacctgcgcgagttcgtgttcaagaacatcgacggctacttcaagatctacagcaagcacacccccatcaacctcgtgcgggacctgccccagggcttcagcgccctggaacccctggtggacctgcccatcggcatcaacatcacccggttccagacactgctggccctgcacagaagctacctgacacccggcgacagcagcagcggatggacagccggcgccgccgcctactacgtgggctacctgcagcccagaaccttcctgctgaagtacaacgagaacggcaccatcaccgacgccgtggactgcgccctggaccccctgagcgagacaaagtgcaccctgaagtccttcaccgtggaaaagggcatctaccagaccagcaacttccgggtgcagcccaccgaaagcatcgtgcggttccccaacatcaccaacctgtgccccttcggcgaggtgttcaacgccaccagattcgccagcgtgtacgcctggaaccggaagcggatcagcaactgcgtggccgactacagcgtgctgtacaacagcgccagcttcagcaccttcaagtgctacggcgtgagccccaccaagctgaacgacctgtgcttcacaaacgtgtacgccgacagcttcgtgatccggggagacgaagtgcggcagatcgcccccggacagacaggcaagatcgccgactacaactacaagctgcccgacgacttcaccggctgcgtgatcgcctggaacagcaacaacctggacagcaaagtcggcggcaactacaactacctgtaccggctgttccggaagtccaacctgaagcccttcgagcgggacatcagcaccgagatctaccaggccggcagcaccccctgcaacggcgtggaaggcttcaactgctacttcccactgcagagctacggcttccagcccacaaacggcgtgggctaccagccctacagagtggtggtgctgagcttcgaactgctgcacgcccccgccacagtgtgcggccccaagaaaagcaccaacctcgtgaagaacaaatgcgtgaacttcaacttcaacggcctgaccggcaccggcgtgctgacagagagcaacaagaagttcctgccattccagcagttcggccgggacatcgccgacaccacagacgccgtcagagacccccagacactggaaatcctggacatcaccccctgcagcttcggcggagtgagcgtgatcacccccggcaccaacaccagcaaccaggtggcagtgctgtaccaggacgtgaactgcaccgaagtgcccgtggccatccacgccgaccagctgacacccacatggcgggtgtacagcaccggcagcaacgtgttccagaccagagccggctgcctgatcggagccgagcacgtgaacaacagctacgagtgcgacatccccatcggcgccggcatctgcgccagctaccagacacagacaaacagccccagacgggccagaagcgtggccagccagagcatcatcgcctacacaatgagcctgggcgccgagaacagcgtggcctacagcaacaacagcatcgccatccccaccaacttcaccatcagcgtgaccacagagatcctgcccgtgagcatgaccaagaccagcgtggactgcaccatgtacatctgcggcgacagcaccgagtgcagcaacctgctgctgcagtacggcagcttctgcacccagctgaacagagccctgacagggatcgccgtggaacaggacaagaacacccaagaggtgttcgcccaagtgaagcagatctacaagaccccccccatcaaggacttcggcggcttcaacttcagccagatcctgcccgaccccagcaagcccagcaagcggagcttcatcgaggacctgctgttcaacaaagtgacactggccgacgccggcttcatcaagcagtacggcgactgcctgggcgacatcgccgccagggacctgatctgcgcccagaagttcaacggactgacagtgctgccccccctgctgaccgacgagatgatcgcccagtacacaagcgccctgctggccggcacaatcacaagcggctggacattcggagccggcgccgccctgcagatccccttcgccatgcagatggcctaccggttcaacggcatcggagtgacccagaacgtgctgtacgagaaccagaagctgatcgccaaccagttcaacagcgccatcggcaagatccaggacagcctgagcagcacagcaagcgccctgggaaagctgcaggacgtggtcaaccagaacgcccaggcactgaacaccctggtcaagcagctgagcagcaacttcggcgccatcagcagcgtgctgaacgacatcctgagcagactggacaaggtggaagccgaggtgcagatcgacagactgatcaccggaaggctgcagagcctgcagacctacgtcacccagcagctgatcagagccgccgagatcagagccagcgccaacctggccgccaccaagatgagcgagtgcgtgctgggccagagcaagagagtggacttctgcggcaagggctaccacctgatgagcttcccccagagcgccccccacggcgtggtgttcctgcacgtgacatacgtgcccgcccaagagaagaacttcaccaccgccccagccatctgccacgacggcaaagcccacttccccagagaaggcgtgttcgtgagcaacggcacccactggttcgtgacccagcggaacttctacgagccccagatcatcaccaccgacaacaccttcgtgagcggcaactgcgacgtcgtgatcggcatcgtgaacaacaccgtgtacgaccccctgcagcccgagctggacagcttcaaagaggaactggacaagtacttcaagaaccacacaagccccgacgtggacctgggcgacatcagcggaatcaacgccagcgtcgtgaacatccagaaagagatcgaccggctgaacgaggtggccaagaacctgaacgagagcctgatcgacctgcaagaactggggaagtacgagcagtacatcaagtggccctggtacatctggctgggcttcatcgccggactgatcgccatcgtgatggtcacaatcatgctgtgctgcatgaccagctgctgcagctgcctgaagggctgctgcagctgcggcagctgctgcaagttcgacgaggacgacagcgagcccgtgctgaagggcgtgaaactgcactacacatgagctcgctttcttgctgtccaatttctattaaaggttcctttgttccctaagtccaactactaaactgggggatattatgaagggccttgagcatctggattctgcctaataaaaaacatttattttcattgcgaattc

SEQ ID NO: 13 - DNA, 30 bp, Artificial Sequence
  primer
tgatgctagcgtaatacgactcactataag

SEQ ID NO: 14 - DNA, 150 bp, Artificial Sequence
  primer
gccaaagcttgctcttcgttttttttttttttttttttttttttttttttttttttttttttttttttttttttttttttttttttttttttttttttttttttttttttttttttttttttttttttgcaatgaaaataaatgtttttt

SEQ ID NO: 15 - DNA, 4180 bp, Artificial Sequence
  template DNA
tgatgctagcgtaatacgactcactataaggagacccaagctacatttgcttctgacacaactgtgttcactagcaacctcaaacagacaccgccaccatgttcgtgttcctggtgctgctgcccctggtgagcagccagtgcgtgaacctgaccaccagaacacagctgcccccagcctacaccaacagcttcaccagaggcgtgtactaccccgacaaggtgttcagaagcagcgtgctgcacagcacccaggacctgttcctgcccttcttcagcaacgtgacctggttccacgccatccacgtgagcggcaccaacggcaccaagagattcgacaaccccgtgctgcccttcaacgacggggtgtacttcgccagcaccgagaagtccaacatcatcagaggctggatcttcggcaccacactggacagcaagacccagagcctgctgatcgtgaacaacgccaccaacgtggtcatcaaagtgtgcgagttccagttctgcaacgaccccttcctgggcgtctactaccacaagaacaacaagagctggatggaaagcgagttccgggtgtacagcagcgccaacaactgcaccttcgagtacgtgagccagcccttcctgatggacctggaaggcaagcagggcaacttcaagaacctgcgcgagttcgtgttcaagaacatcgacggctacttcaagatctacagcaagcacacccccatcaacctcgtgcgggacctgccccagggcttcagcgccctggaacccctggtggacctgcccatcggcatcaacatcacccggttccagacactgctggccctgcacagaagctacctgacacccggcgacagcagcagcggatggacagccggcgccgccgcctactacgtgggctacctgcagcccagaaccttcctgctgaagtacaacgagaacggcaccatcaccgacgccgtggactgcgccctggaccccctgagcgagacaaagtgcaccctgaagtccttcaccgtggaaaagggcatctaccagaccagcaacttccgggtgcagcccaccgaaagcatcgtgcggttccccaacatcaccaacctgtgccccttcggcgaggtgttcaacgccaccagattcgccagcgtgtacgcctggaaccggaagcggatcagcaactgcgtggccgactacagcgtgctgtacaacagcgccagcttcagcaccttcaagtgctacggcgtgagccccaccaagctgaacgacctgtgcttcacaaacgtgtacgccgacagcttcgtgatccggggagacgaagtgcggcagatcgcccccggacagacaggcaagatcgccgactacaactacaagctgcccgacgacttcaccggctgcgtgatcgcctggaacagcaacaacctggacagcaaagtcggcggcaactacaactacctgtaccggctgttccggaagtccaacctgaagcccttcgagcgggacatcagcaccgagatctaccaggccggcagcaccccctgcaacggcgtggaaggcttcaactgctacttcccactgcagagctacggcttccagcccacaaacggcgtgggctaccagccctacagagtggtggtgctgagcttcgaactgctgcacgcccccgccacagtgtgcggccccaagaaaagcaccaacctcgtgaagaacaaatgcgtgaacttcaacttcaacggcctgaccggcaccggcgtgctgacagagagcaacaagaagttcctgccattccagcagttcggccgggacatcgccgacaccacagacgccgtcagagacccccagacactggaaatcctggacatcaccccctgcagcttcggcggagtgagcgtgatcacccccggcaccaacaccagcaaccaggtggcagtgctgtaccaggacgtgaactgcaccgaagtgcccgtggccatccacgccgaccagctgacacccacatggcgggtgtacagcaccggcagcaacgtgttccagaccagagccggctgcctgatcggagccgagcacgtgaacaacagctacgagtgcgacatccccatcggcgccggcatctgcgccagctaccagacacagacaaacagccccagacgggccagaagcgtggccagccagagcatcatcgcctacacaatgagcctgggcgccgagaacagcgtggcctacagcaacaacagcatcgccatccccaccaacttcaccatcagcgtgaccacagagatcctgcccgtgagcatgaccaagaccagcgtggactgcaccatgtacatctgcggcgacagcaccgagtgcagcaacctgctgctgcagtacggcagcttctgcacccagctgaacagagccctgacagggatcgccgtggaacaggacaagaacacccaagaggtgttcgcccaagtgaagcagatctacaagaccccccccatcaaggacttcggcggcttcaacttcagccagatcctgcccgaccccagcaagcccagcaagcggagcttcatcgaggacctgctgttcaacaaagtgacactggccgacgccggcttcatcaagcagtacggcgactgcctgggcgacatcgccgccagggacctgatctgcgcccagaagttcaacggactgacagtgctgccccccctgctgaccgacgagatgatcgcccagtacacaagcgccctgctggccggcacaatcacaagcggctggacattcggagccggcgccgccctgcagatccccttcgccatgcagatggcctaccggttcaacggcatcggagtgacccagaacgtgctgtacgagaaccagaagctgatcgccaaccagttcaacagcgccatcggcaagatccaggacagcctgagcagcacagcaagcgccctgggaaagctgcaggacgtggtcaaccagaacgcccaggcactgaacaccctggtcaagcagctgagcagcaacttcggcgccatcagcagcgtgctgaacgacatcctgagcagactggacaaggtggaagccgaggtgcagatcgacagactgatcaccggaaggctgcagagcctgcagacctacgtcacccagcagctgatcagagccgccgagatcagagccagcgccaacctggccgccaccaagatgagcgagtgcgtgctgggccagagcaagagagtggacttctgcggcaagggctaccacctgatgagcttcccccagagcgccccccacggcgtggtgttcctgcacgtgacatacgtgcccgcccaagagaagaacttcaccaccgccccagccatctgccacgacggcaaagcccacttccccagagaaggcgtgttcgtgagcaacggcacccactggttcgtgacccagcggaacttctacgagccccagatcatcaccaccgacaacaccttcgtgagcggcaactgcgacgtcgtgatcggcatcgtgaacaacaccgtgtacgaccccctgcagcccgagctggacagcttcaaagaggaactggacaagtacttcaagaaccacacaagccccgacgtggacctgggcgacatcagcggaatcaacgccagcgtcgtgaacatccagaaagagatcgaccggctgaacgaggtggccaagaacctgaacgagagcctgatcgacctgcaagaactggggaagtacgagcagtacatcaagtggccctggtacatctggctgggcttcatcgccggactgatcgccatcgtgatggtcacaatcatgctgtgctgcatgaccagctgctgcagctgcctgaagggctgctgcagctgcggcagctgctgcaagttcgacgaggacgacagcgagcccgtgctgaagggcgtgaaactgcactacacatgagctcgctttcttgctgtccaatttctattaaaggttcctttgttccctaagtccaactactaaactgggggatattatgaagggccttgagcatctggattctgcctaataaaaaacatttattttcattgcaaaaaaaaaaaaaaaaaaaaaaaaaaaaaaaaaaaaaaaaaaaaaaaaaaaaaaaaaaaaaaaaaaaaaaaaaaaaaaaaaaaaaaaaaaaaaaaaaaaaaaaaaaaaaacgaagagcaagctttggc

SEQ ID NO: 16 - RNA, 4134 nt, Artificial Sequence
  SARS-CoV-2 S full optimized mRNA-003
aggagacccaagcuacauuugcuucugacacaacuguguucacuagcaaccucaaacagacaccgccaccauguucguguuccuggugcugcugccccuggugagcagccagugcgugaaccugaccaccagaacacagcugcccccagccuacaccaacagcuucaccagaggcguguacuaccccgacaagguguucagaagcagcgugcugcacagcacccaggaccuguuccugcccuucuucagcaacgugaccugguuccacgccauccacgugagcggcaccaacggcaccaagagauucgacaaccccgugcugcccuucaacgacgggguguacuucgccagcaccgagaaguccaacaucaucagaggcuggaucuucggcaccacacuggacagcaagacccagagccugcugaucgugaacaacgccaccaacguggucaucaaagugugcgaguuccaguucugcaacgaccccuuccugggcgucuacuaccacaagaacaacaagagcuggauggaaagcgaguuccggguguacagcagcgccaacaacugcaccuucgaguacgugagccagcccuuccugauggaccuggaaggcaagcagggcaacuucaagaaccugcgcgaguucguguucaagaacaucgacggcuacuucaagaucuacagcaagcacacccccaucaaccucgugcgggaccugccccagggcuucagcgcccuggaaccccugguggaccugcccaucggcaucaacaucacccgguuccagacacugcuggcccugcacagaagcuaccugacacccggcgacagcagcagcggauggacagccggcgccgccgccuacuacgugggcuaccugcagcccagaaccuuccugcugaaguacaacgagaacggcaccaucaccgacgccguggacugcgcccuggacccccugagcgagacaaagugcacccugaaguccuucaccguggaaaagggcaucuaccagaccagcaacuuccgggugcagcccaccgaaagcaucgugcgguuccccaacaucaccaaccugugccccuucggcgagguguucaacgccaccagauucgccagcguguacgccuggaaccggaagcggaucagcaacugcguggccgacuacagcgugcuguacaacagcgccagcuucagcaccuucaagugcuacggcgugagccccaccaagcugaacgaccugugcuucacaaacguguacgccgacagcuucgugauccggggagacgaagugcggcagaucgcccccggacagacaggcaagaucgccgacuacaacuacaagcugcccgacgacuucaccggcugcgugaucgccuggaacagcaacaaccuggacagcaaagucggcggcaacuacaacuaccuguaccggcuguuccggaaguccaaccugaagcccuucgagcgggacaucagcaccgagaucuaccaggccggcagcacccccugcaacggcguggaaggcuucaacugcuacuucccacugcagagcuacggcuuccagcccacaaacggcgugggcuaccagcccuacagagugguggugcugagcuucgaacugcugcacgcccccgccacagugugcggccccaagaaaagcaccaaccucgugaagaacaaaugcgugaacuucaacuucaacggccugaccggcaccggcgugcugacagagagcaacaagaaguuccugccauuccagcaguucggccgggacaucgccgacaccacagacgccgucagagacccccagacacuggaaauccuggacaucacccccugcagcuucggcggagugagcgugaucacccccggcaccaacaccagcaaccagguggcagugcuguaccaggacgugaacugcaccgaagugcccguggccauccacgccgaccagcugacacccacauggcggguguacagcaccggcagcaacguguuccagaccagagccggcugccugaucggagccgagcacgugaacaacagcuacgagugcgacauccccaucggcgccggcaucugcgccagcuaccagacacagacaaacagccccagacgggccagaagcguggccagccagagcaucaucgccuacacaaugagccugggcgccgagaacagcguggccuacagcaacaacagcaucgccauccccaccaacuucaccaucagcgugaccacagagauccugcccgugagcaugaccaagaccagcguggacugcaccauguacaucugcggcgacagcaccgagugcagcaaccugcugcugcaguacggcagcuucugcacccagcugaacagagcccugacagggaucgccguggaacaggacaagaacacccaagagguguucgcccaagugaagcagaucuacaagaccccccccaucaaggacuucggcggcuucaacuucagccagauccugcccgaccccagcaagcccagcaagcggagcuucaucgaggaccugcuguucaacaaagugacacuggccgacgccggcuucaucaagcaguacggcgacugccugggcgacaucgccgccagggaccugaucugcgcccagaaguucaacggacugacagugcugcccccccugcugaccgacgagaugaucgcccaguacacaagcgcccugcuggccggcacaaucacaagcggcuggacauucggagccggcgccgcccugcagauccccuucgccaugcagauggccuaccgguucaacggcaucggagugacccagaacgugcuguacgagaaccagaagcugaucgccaaccaguucaacagcgccaucggcaagauccaggacagccugagcagcacagcaagcgcccugggaaagcugcaggacguggucaaccagaacgcccaggcacugaacacccuggucaagcagcugagcagcaacuucggcgccaucagcagcgugcugaacgacauccugagcagacuggacaagguggaagccgaggugcagaucgacagacugaucaccggaaggcugcagagccugcagaccuacgucacccagcagcugaucagagccgccgagaucagagccagcgccaaccuggccgccaccaagaugagcgagugcgugcugggccagagcaagagaguggacuucugcggcaagggcuaccaccugaugagcuucccccagagcgccccccacggcgugguguuccugcacgugacauacgugcccgcccaagagaagaacuucaccaccgccccagccaucugccacgacggcaaagcccacuuccccagagaaggcguguucgugagcaacggcacccacugguucgugacccagcggaacuucuacgagccccagaucaucaccaccgacaacaccuucgugagcggcaacugcgacgucgugaucggcaucgugaacaacaccguguacgacccccugcagcccgagcuggacagcuucaaagaggaacuggacaaguacuucaagaaccacacaagccccgacguggaccugggcgacaucagcggaaucaacgccagcgucgugaacauccagaaagagaucgaccggcugaacgagguggccaagaaccugaacgagagccugaucgaccugcaagaacuggggaaguacgagcaguacaucaaguggcccugguacaucuggcugggcuucaucgccggacugaucgccaucgugauggucacaaucaugcugugcugcaugaccagcugcugcagcugccugaagggcugcugcagcugcggcagcugcugcaaguucgacgaggacgacagcgagcccgugcugaagggcgugaaacugcacuacacaugagcucgcuuucuugcuguccaauuucuauuaaagguuccuuuguucccuaaguccaacuacuaaacugggggauauuaugaagggccuugagcaucuggauucugccuaauaaaaaacauuuauuuucauugcaaaaaaaaaaaaaaaaaaaaaaaaaaaaaaaaaaaaaaaaaaaaaaaaaaaaaaaaaaaaaaaaaaaaaaaaaaaaaaaaaaaaaaaaaaaaaaaaaaaaaaaaaaaaaa

SEQ ID NO: 17 - DNA, 943 bp, Artificial Sequence
  DNA insert
gctagcgtaatacgactcactataaggagacccaagctacatttgcttctgacacaactgtgttcactagcaacctcaaacagacaccgccaccatgttcgtgttcctggtgctgctgcccctggtgagcagcagagtgcagcccaccgagagcatcgtgcggttccccaacatcaccaacctgtgccccttcggcgaggtgttcaacgccaccagattcgccagcgtgtacgcctggaaccggaagcggatcagcaactgcgtggccgactacagcgtgctgtacaacagcgccagcttcagcaccttcaagtgctacggcgtgagccccaccaagctgaacgacctgtgcttcaccaacgtgtacgccgacagcttcgtgatcagaggcgacgaagtgcggcagatcgcccccggacagacaggcaagatcgccgactacaactacaagctgcccgacgacttcaccggctgcgtgatcgcctggaacagcaacaacctggacagcaaagtcggcggcaactacaactacctgtaccggctgttccggaagtccaacctgaagcccttcgagcgggacatcagcaccgagatctaccaggccggcagcaccccctgcaacggcgtggaaggcttcaactgctacttcccactgcagagctacggcttccagcccacaaacggcgtgggctaccagccctacagagtggtggtgctgagcttcgagctgctgcacgcccccgccacagtgtgcggccccaagaaaagcaccaacctggtcaagaacaaatgcgtgaacttctgagctcgctttcttgctgtccaatttctattaaaggttcctttgttccctaagtccaactactaaactgggggatattatgaagggccttgagcatctggattctgcctaataaaaaacatttattttcattgcgaattc

SEQ ID NO: 18 - DNA, 1069 bp, Artificial Sequence
  template DNA
tgatgctagcgtaatacgactcactataaggagacccaagctacatttgcttctgacacaactgtgttcactagcaacctcaaacagacaccgccaccatgttcgtgttcctggtgctgctgcccctggtgagcagcagagtgcagcccaccgagagcatcgtgcggttccccaacatcaccaacctgtgccccttcggcgaggtgttcaacgccaccagattcgccagcgtgtacgcctggaaccggaagcggatcagcaactgcgtggccgactacagcgtgctgtacaacagcgccagcttcagcaccttcaagtgctacggcgtgagccccaccaagctgaacgacctgtgcttcaccaacgtgtacgccgacagcttcgtgatcagaggcgacgaagtgcggcagatcgcccccggacagacaggcaagatcgccgactacaactacaagctgcccgacgacttcaccggctgcgtgatcgcctggaacagcaacaacctggacagcaaagtcggcggcaactacaactacctgtaccggctgttccggaagtccaacctgaagcccttcgagcgggacatcagcaccgagatctaccaggccggcagcaccccctgcaacggcgtggaaggcttcaactgctacttcccactgcagagctacggcttccagcccacaaacggcgtgggctaccagccctacagagtggtggtgctgagcttcgagctgctgcacgcccccgccacagtgtgcggccccaagaaaagcaccaacctggtcaagaacaaatgcgtgaacttctgagctcgctttcttgctgtccaatttctattaaaggttcctttgttccctaagtccaactactaaactgggggatattatgaagggccttgagcatctggattctgcctaataaaaaacatttattttcattgcaaaaaaaaaaaaaaaaaaaaaaaaaaaaaaaaaaaaaaaaaaaaaaaaaaaaaaaaaaaaaaaaaaaaaaaaaaaaaaaaaaaaaaaaaaaaaaaaaaaaaaaaaaaaaacgaagagcaagctttggc

SEQ ID NO: 19 - RNA, 1023 nt, Artificial Sequence
  SARS-CoV-2 RBD optimized mRNA-004
aggagacccaagcuacauuugcuucugacacaacuguguucacuagcaaccucaaacagacaccgccaccauguucguguuccuggugcugcugccccuggugagcagcagagugcagcccaccgagagcaucgugcgguuccccaacaucaccaaccugugccccuucggcgagguguucaacgccaccagauucgccagcguguacgccuggaaccggaagcggaucagcaacugcguggccgacuacagcgugcuguacaacagcgccagcuucagcaccuucaagugcuacggcgugagccccaccaagcugaacgaccugugcuucaccaacguguacgccgacagcuucgugaucagaggcgacgaagugcggcagaucgcccccggacagacaggcaagaucgccgacuacaacuacaagcugcccgacgacuucaccggcugcgugaucgccuggaacagcaacaaccuggacagcaaagucggcggcaacuacaacuaccuguaccggcuguuccggaaguccaaccugaagcccuucgagcgggacaucagcaccgagaucuaccaggccggcagcacccccugcaacggcguggaaggcuucaacugcuacuucccacugcagagcuacggcuuccagcccacaaacggcgugggcuaccagcccuacagagugguggugcugagcuucgagcugcugcacgcccccgccacagugugcggccccaagaaaagcaccaaccuggucaagaacaaaugcgugaacuucugagcucgcuuucuugcuguccaauuucuauuaaagguuccuuuguucccuaaguccaacuacuaaacugggggauauuaugaagggccuugagcaucuggauucugccuaauaaaaaacauuuauuuucauugcaaaaaaaaaaaaaaaaaaaaaaaaaaaaaaaaaaaaaaaaaaaaaaaaaaaaaaaaaaaaaaaaaaaaaaaaaaaaaaaaaaaaaaaaaaaaaaaaaaaaaaaaaaaaaa

SEQ ID NO: 20 - DNA, 995 bp, Artificial Sequence
  template DNA
gctagcgtaatacgactcactataaggagacccaagctacatttgcttctgacacaactgtgttcactagcaacctcaaacagacaccgccaccatgttcgtgttcctggtgctgctgcccctggtgagcagcagagtgcagcccaccgagagcatcgtgcggttccccaacatcaccaacctgtgccccttcggcgaggtgttcaacgccaccagattcgccagcgtgtacgcctggaaccggaagcggatcagcaactgcgtggccgactacagcgtgctgtacaacagcgccagcttcagcaccttcaagtgctacggcgtgagccccaccaagctgaacgacctgtgcttcaccaacgtgtacgccgacagcttcgtgatcagaggcgacgaagtgcggcagatcgcccccggacagacaggcaagatcgccgactacaactacaagctgcccgacgacttcaccggctgcgtgatcgcctggaacagcaacaacctggacagcaaagtcggcggcaactacaactacctgtaccggctgttccggaaaagcaacctgaagcccttcgagcgggacatcagcaccgagatctaccaggccggcagcaccccctgcaacggcgtggaaggcttcaactgctacttcccactgcagagctacggcttccagcccacaaacggcgtgggctaccagccctacagagtggtggtgctgagcttcgagctgctgcacgcccccgccacagtgtgcggccccaagaaaagcaccaacctggtcaagaacaaatgcgtgaacttctgagctcgctttcttgctgtccaatttctattaaaggttcctttgttccctaagtccaactactaaactgggggatattatgaagggccttgagcatctggattctgcctaataaaaaacatttattttcattgcaaaaaaaaaaaaaaaaaaaaaaaaaaaaaaaaaaaaaaaaaaaaaaaaaacgaagagc

SEQ ID NO: 21 - RNA, 963 nt, Artificial Sequence
  SARS-CoV-2 RBD S2000 mRNA
aggagacccaagcuacauuugcuucugacacaacuguguucacuagcaaccucaaacagacaccgccaccauguucguguuccuggugcugcugccccuggugagcagcagagugcagcccaccgagagcaucgugcgguuccccaacaucaccaaccugugccccuucggcgagguguucaacgccaccagauucgccagcguguacgccuggaaccggaagcggaucagcaacugcguggccgacuacagcgugcuguacaacagcgccagcuucagcaccuucaagugcuacggcgugagccccaccaagcugaacgaccugugcuucaccaacguguacgccgacagcuucgugaucagaggcgacgaagugcggcagaucgcccccggacagacaggcaagaucgccgacuacaacuacaagcugcccgacgacuucaccggcugcgugaucgccuggaacagcaacaaccuggacagcaaagucggcggcaacuacaacuaccuguaccggcuguuccggaaaagcaaccugaagcccuucgagcgggacaucagcaccgagaucuaccaggccggcagcacccccugcaacggcguggaaggcuucaacugcuacuucccacugcagagcuacggcuuccagcccacaaacggcgugggcuaccagcccuacagagugguggugcugagcuucgagcugcugcacgcccccgccacagugugcggccccaagaaaagcaccaaccuggucaagaacaaaugcgugaacuucugagcucgcuuucuugcuguccaauuucuauuaaagguuccuuuguucccuaaguccaacuacuaaacugggggauauuaugaagggccuugagcaucuggauucugccuaauaaaaaacauuuauuuucauugcaaaaaaaaaaaaaaaaaaaaaaaaaaaaaaaaaaaaaaaaaaaaaaaaaa

SEQ ID NO: 22 - DNA, 995 bp, Artificial Sequence
  template DNA
gctagcgtaatacgactcactataaggagacccaagctacatttgcttctgacacaactgtgttcactagcaacctcaaacagacaccgccaccatgttcgtgttcctggtgctgctgcccctggtgagcagcagagtgcagcccaccgagagcatcgtgcggttccccaacatcaccaacctgtgccccttcggcgaggtgttcaacgccaccagattcgccagcgtgtacgcctggaaccggaagcggatcagcaactgcgtggccgactacagcgtgctgtacaacagcgccagcttcagcaccttcaagtgctacggcgtgagccccaccaagctgaacgacctgtgcttcaccaacgtgtacgccgacagcttcgtgatcagaggcgacgaagtgcggcagatcgcccccggacagacaggcaagatcgccgactacaactacaagctgcccgacgacttcaccggctgcgtgatcgcctggaacagcaacaacctggacagcaaagtcggcggcaactacaactacctgtaccggctgttccggaaaagcaacctgaagcccttcgagcgggacatcagcaccgagatctaccaggccggcagcaccccctgcaacggcgtggaaggcttcaactgctacttcccactgcagagctacggcttccagcccacaaacggcgtgggctaccagccctacagagtggtggtgctgagcttcgagctgctgcacgcccccgccacagtgtgcggccccaagaaaagcaccaacctggtcaagaacaagagcgtgaacttctgagctcgctttcttgctgtccaatttctattaaaggttcctttgttccctaagtccaactactaaactgggggatattatgaagggccttgagcatctggattctgcctaataaaaaacatttattttcattgcaaaaaaaaaaaaaaaaaaaaaaaaaaaaaaaaaaaaaaaaaaaaaaaaaacgaagagc

SEQ ID NO: 23 - RNA, 963 nt, Artificial Sequence
  SARS-CoV-2 RBD S2001 mRNA
aggagacccaagcuacauuugcuucugacacaacuguguucacuagcaaccucaaacagacaccgccaccauguucguguuccuggugcugcugccccuggugagcagcagagugcagcccaccgagagcaucgugcgguuccccaacaucaccaaccugugccccuucggcgagguguucaacgccaccagauucgccagcguguacgccuggaaccggaagcggaucagcaacugcguggccgacuacagcgugcuguacaacagcgccagcuucagcaccuucaagugcuacggcgugagccccaccaagcugaacgaccugugcuucaccaacguguacgccgacagcuucgugaucagaggcgacgaagugcggcagaucgcccccggacagacaggcaagaucgccgacuacaacuacaagcugcccgacgacuucaccggcugcgugaucgccuggaacagcaacaaccuggacagcaaagucggcggcaacuacaacuaccuguaccggcuguuccggaaaagcaaccugaagcccuucgagcgggacaucagcaccgagaucuaccaggccggcagcacccccugcaacggcguggaaggcuucaacugcuacuucccacugcagagcuacggcuuccagcccacaaacggcgugggcuaccagcccuacagagugguggugcugagcuucgagcugcugcacgcccccgccacagugugcggccccaagaaaagcaccaaccuggucaagaacaagagcgugaacuucugagcucgcuuucuugcuguccaauuucuauuaaagguuccuuuguucccuaaguccaacuacuaaacugggggauauuaugaagggccuugagcaucuggauucugccuaauaaaaaacauuuauuuucauugcaaaaaaaaaaaaaaaaaaaaaaaaaaaaaaaaaaaaaaaaaaaaaaaaaa

SEQ ID NO: 24 - protein, 236 aa, Artificial Sequence
  spike protein signal sequence added SARS-CoV-2 RBD S2001
MFVFLVLLPLVSSRVQPTESIVRFPNITNLCPFGEVFNATRFASVYAWNRKRISNCVADYSVLYNSASFSTFKCYGVSPTKLNDLCFTNVYADSFVIRGDEVRQIAPGQTGKIADYNYKLPDDFTGCVIAWNSNNLDSKVGGNYNYLYRLFRKSNLKPFERDISTEIYQAGSTPCNGVEGFNCYFPLQSYGFQPTNGVGYQPYRVVVLSFELLHAPATVCGPKKSTNLVKNKSVNF

SEQ ID NO: 25 - protein, 223 aa, Artificial Sequence
  SARS-CoV-2 RBD S2001
RVQPTESIVRFPNITNLCPFGEVFNATRFASVYAWNRKRISNCVADYSVLYNSASFSTFKCYGVSPTKLNDLCFTNVYADSFVIRGDEVRQIAPGQTGKIADYNYKLPDDFTGCVIAWNSNNLDSKVGGNYNYLYRLFRKSNLKPFERDISTEIYQAGSTPCNGVEGFNCYFPLQSYGFQPTNGVGYQPYRVVVLSFELLHAPATVCGPKKSTNLVKNKSVNF

SEQ ID NO: 26 - DNA, 926 bp, Artificial Sequence
  template DNA
gctagcgtaatacgactcactataaggagacccaagctacatttgcttctgacacaactgtgttcactagcaacctcaaacagacaccgccaccatgttcgtgttcctggtgctgctgcccctggtgagcagcttccccaacatcaccaacctgtgccccttcggcgaggtgttcaacgccacaagattcgccagcgtgtacgcctggaaccggaagcggatcagcaactgcgtggccgactacagcgtgctgtacaacagcgccagcttcagcaccttcaagtgctacggcgtgagccccaccaagctgaacgacctgtgcttcaccaacgtgtacgccgacagcttcgtgatcagaggcgacgaagtgcggcagatcgcccccggacagacaggcaagatcgccgactacaactacaagctgcccgacgacttcaccggctgcgtgatcgcctggaacagcaacaacctggacagcaaagtcggcggcaactacaactacctgtaccggctgttccggaaaagcaacctgaagcccttcgagcgggacatcagcaccgagatctaccaggccggcagcaccccctgcaacggcgtggaaggcttcaactgctacttcccactgcagagctacggcttccagcccacaaacggcgtgggctaccagccctacagagtggtggtgctgagcttcgagctgctgcacgcccccgccacagtgtgcggacccaaatgagctcgctttcttgctgtccaatttctattaaaggttcctttgttccctaagtccaactactaaactgggggatattatgaagggccttgagcatctggattctgcctaataaaaaacatttattttcattgcaaaaaaaaaaaaaaaaaaaaaaaaaaaaaaaaaaaaaaaaaaaaaaaaaacgaagagc

SEQ ID NO: 27 - RNA, 894 nt, Artificial Sequence
  SARS-CoV-2 RBD S2002 mRNA
aggagacccaagcuacauuugcuucugacacaacuguguucacuagcaaccucaaacagacaccgccaccauguucguguuccuggugcugcugccccuggugagcagcuuccccaacaucaccaaccugugccccuucggcgagguguucaacgccacaagauucgccagcguguacgccuggaaccggaagcggaucagcaacugcguggccgacuacagcgugcuguacaacagcgccagcuucagcaccuucaagugcuacggcgugagccccaccaagcugaacgaccugugcuucaccaacguguacgccgacagcuucgugaucagaggcgacgaagugcggcagaucgcccccggacagacaggcaagaucgccgacuacaacuacaagcugcccgacgacuucaccggcugcgugaucgccuggaacagcaacaaccuggacagcaaagucggcggcaacuacaacuaccuguaccggcuguuccggaaaagcaaccugaagcccuucgagcgggacaucagcaccgagaucuaccaggccggcagcacccccugcaacggcguggaaggcuucaacugcuacuucccacugcagagcuacggcuuccagcccacaaacggcgugggcuaccagcccuacagagugguggugcugagcuucgagcugcugcacgcccccgccacagugugcggacccaaaugagcucgcuuucuugcuguccaauuucuauuaaagguuccuuuguucccuaaguccaacuacuaaacugggggauauuaugaagggccuugagcaucuggauucugccuaauaaaaaacauuuauuuucauugcaaaaaaaaaaaaaaaaaaaaaaaaaaaaaaaaaaaaaaaaaaaaaaaaaa

SEQ ID NO: 28 - protein, 213 aa, Artificial Sequence
  spike protein signal sequence added SARS-CoV-2 RBD S2002
MFVFLVLLPLVSSFPNITNLCPFGEVFNATRFASVYAWNRKRISNCVADYSVLYNSASFSTFKCYGVSPTKLNDLCFTNVYADSFVIRGDEVRQIAPGQTGKIADYNYKLPDDFTGCVIAWNSNNLDSKVGGNYNYLYRLFRKSNLKPFERDISTEIYQAGSTPCNGVEGFNCYFPLQSYGFQPTNGVGYQPYRVVVLSFELLHAPATVCGPK

SEQ ID NO: 29 - protein, 200 aa, Artificial Sequence
  SARS-CoV-2 RBD S2002
FPNITNLCPFGEVFNATRFASVYAWNRKRISNCVADYSVLYNSASFSTFKCYGVSPTKLNDLCFTNVYADSFVIRGDEVRQIAPGQTGKIADYNYKLPDDFTGCVIAWNSNNLDSKVGGNYNYLYRLFRKSNLKPFERDISTEIYQAGSTPCNGVEGFNCYFPLQSYGFQPTNGVGYQPYRVVVLSFELLHAPATVCGPK

SEQ ID NO: 30 - DNA, 1064 bp, Artificial Sequence
  template DNA
gctagcgtaatacgactcactataaggagacccaagctacatttgcttctgacacaactgtgttcactagcaacctcaaacagacaccgccaccatgttcgtgttcctggtgctgctgcccctggtgagcagcgagaagggcatctaccagaccagcaacttcagagtgcagcccaccgagagcatcgtgcggttccccaacatcaccaacctgtgccccttcggcgaggtgttcaacgccaccagattcgccagcgtgtacgcctggaaccggaagcggatcagcaactgcgtggccgactacagcgtgctgtacaacagcgccagcttcagcaccttcaagtgctacggcgtgagccccaccaagctgaacgacctgtgcttcaccaacgtgtacgccgacagcttcgtgatcagaggcgacgaagtgcggcagatcgcccccggacagacaggcaagatcgccgactacaactacaagctgcccgacgacttcaccggctgcgtgatcgcctggaacagcaacaacctggacagcaaagtcggcggcaactacaactacctgtaccggctgttccggaaaagcaacctgaagcccttcgagcgggacatcagcaccgagatctaccaggccggcagcaccccctgcaacggcgtggaaggcttcaactgctacttcccactgcagagctacggcttccagcccacaaacggcgtgggctaccagccctacagagtggtggtgctgagcttcgagctgctgcacgcccccgccacagtgtgcggccccaagaaaagcaccaacctggtcaagaacaagagcgtgaacttcaacttcaacggcctgaccggcaccggcgtgttgacagaatgagctcgctttcttgctgtccaatttctattaaaggttcctttgttccctaagtccaactactaaactgggggatattatgaagggccttgagcatctggattctgcctaataaaaaacatttattttcattgcaaaaaaaaaaaaaaaaaaaaaaaaaaaaaaaaaaaaaaaaaaaaaaaaaacgaagagc

SEQ ID NO: 31 - RNA, 1032 nt, Artificial Sequence
  SARS-CoV-2 RBD S2003 mRNA
aggagacccaagcuacauuugcuucugacacaacuguguucacuagcaaccucaaacagacaccgccaccauguucguguuccuggugcugcugccccuggugagcagcgagaagggcaucuaccagaccagcaacuucagagugcagcccaccgagagcaucgugcgguuccccaacaucaccaaccugugccccuucggcgagguguucaacgccaccagauucgccagcguguacgccuggaaccggaagcggaucagcaacugcguggccgacuacagcgugcuguacaacagcgccagcuucagcaccuucaagugcuacggcgugagccccaccaagcugaacgaccugugcuucaccaacguguacgccgacagcuucgugaucagaggcgacgaagugcggcagaucgcccccggacagacaggcaagaucgccgacuacaacuacaagcugcccgacgacuucaccggcugcgugaucgccuggaacagcaacaaccuggacagcaaagucggcggcaacuacaacuaccuguaccggcuguuccggaaaagcaaccugaagcccuucgagcgggacaucagcaccgagaucuaccaggccggcagcacccccugcaacggcguggaaggcuucaacugcuacuucccacugcagagcuacggcuuccagcccacaaacggcgugggcuaccagcccuacagagugguggugcugagcuucgagcugcugcacgcccccgccacagugugcggccccaagaaaagcaccaaccuggucaagaacaagagcgugaacuucaacuucaacggccugaccggcaccggcguguugacagaaugagcucgcuuucuugcuguccaauuucuauuaaagguuccuuuguucccuaaguccaacuacuaaacugggggauauuaugaagggccuugagcaucuggauucugccuaauaaaaaacauuuauuuucauugcaaaaaaaaaaaaaaaaaaaaaaaaaaaaaaaaaaaaaaaaaaaaaaaaaa

SEQ ID NO: 32 - protein, 259 aa, Artificial Sequence
  spike protein signal sequence added SARS-CoV-2 RBD S2003
MFVFLVLLPLVSSEKGIYQTSNFRVQPTESIVRFPNITNLCPFGEVFNATRFASVYAWNRKRISNCVADYSVLYNSASFSTFKCYGVSPTKLNDLCFTNVYADSFVIRGDEVRQIAPGQTGKIADYNYKLPDDFTGCVIAWNSNNLDSKVGGNYNYLYRLFRKSNLKPFERDISTEIYQAGSTPCNGVEGFNCYFPLQSYGFQPTNGVGYQPYRVVVLSFELLHAPATVCGPKKSTNLVKNKSVNFNFNGLTGTGVLTE

SEQ ID NO: 33 - protein, 246 aa, Artificial Sequence
  SARS-CoV-2 RBD S2003
EKGIYQTSNFRVQPTESIVRFPNITNLCPFGEVFNATRFASVYAWNRKRISNCVADYSVLYNSASFSTFKCYGVSPTKLNDLCFTNVYADSFVIRGDEVRQIAPGQTGKIADYNYKLPDDFTGCVIAWNSNNLDSKVGGNYNYLYRLFRKSNLKPFERDISTEIYQAGSTPCNGVEGFNCYFPLQSYGFQPTNGVGYQPYRVVVLSFELLHAPATVCGPKKSTNLVKNKSVNFNFNGLTGTGVLTE

SEQ ID NO: 34 - DNA, 995 bp, Artificial Sequence
  template DNA
gctagcgtaatacgactcactataaggagacccaagctacatttgcttctgacacaactgtgttcactagcaacctcaaacagacaccgccaccatgttcgtgttcctggtgctgctgcccctggtgagcagcagagtgcagcccaccgagagcatcgtgcggttccccaacatcaccaacctgtgccccttcggcgaggtgttcaacgccaccagattcgccagcgtgtacgcctggaaccggaagcggatcaacaactgcgtggccgactacagcgtgctgtacaacagcaccagcttcagcaccttcaagtgctacggcgtgagccccaccaagctgaacgacctgtgcttcaccaacgtgtacgccgacagcttcgtgatcagaggcgacgaagtgcggcagatcgcccccggacagacaggcaagatcgccgactacaactacaagctgcccgacgacttcaccggctgcgtgatcgcctggaacagcaacaccctggacagcaaagtcggcggcaactacacctacctgtaccggctgttcagaaagagcaacctgaagcccttcgagcgggacatcagcaccgagatctaccaggccggcagcaccccctgcaacggcgtggaaggcttcaactgctacttcccactgcagagctacggcttccagcccacaaacggcgtgggctaccagccctacagagtggtggtgctgagcttcgagctgctgcacgcccccgccacagtgtgcggccccaagaaaagcaccaacctggtcaagaacaagagcgtgaacttctgagctcgctttcttgctgtccaatttctattaaaggttcctttgttccctaagtccaactactaaactgggggatattatgaagggccttgagcatctggattctgcctaataaaaaacatttattttcattgcaaaaaaaaaaaaaaaaaaaaaaaaaaaaaaaaaaaaaaaaaaaaaaaaaacgaagagc

SEQ ID NO: 35 - RNA, 963 nt, Artificial Sequence
  SARS-CoV-2 RBD S2004 mRNA
aggagacccaagcuacauuugcuucugacacaacuguguucacuagcaaccucaaacagacaccgccaccauguucguguuccuggugcugcugccccuggugagcagcagagugcagcccaccgagagcaucgugcgguuccccaacaucaccaaccugugccccuucggcgagguguucaacgccaccagauucgccagcguguacgccuggaaccggaagcggaucaacaacugcguggccgacuacagcgugcuguacaacagcaccagcuucagcaccuucaagugcuacggcgugagccccaccaagcugaacgaccugugcuucaccaacguguacgccgacagcuucgugaucagaggcgacgaagugcggcagaucgcccccggacagacaggcaagaucgccgacuacaacuacaagcugcccgacgacuucaccggcugcgugaucgccuggaacagcaacacccuggacagcaaagucggcggcaacuacaccuaccuguaccggcuguucagaaagagcaaccugaagcccuucgagcgggacaucagcaccgagaucuaccaggccggcagcacccccugcaacggcguggaaggcuucaacugcuacuucccacugcagagcuacggcuuccagcccacaaacggcgugggcuaccagcccuacagagugguggugcugagcuucgagcugcugcacgcccccgccacagugugcggccccaagaaaagcaccaaccuggucaagaacaagagcgugaacuucugagcucgcuuucuugcuguccaauuucuauuaaagguuccuuuguucccuaaguccaacuacuaaacugggggauauuaugaagggccuugagcaucuggauucugccuaauaaaaaacauuuauuuucauugcaaaaaaaaaaaaaaaaaaaaaaaaaaaaaaaaaaaaaaaaaaaaaaaaaa

SEQ ID NO: 36 - protein, 236 aa, Artificial Sequence
  spike protein signal sequence added SARS-CoV-2 RBD S2004
MFVFLVLLPLVSSRVQPTESIVRFPNITNLCPFGEVFNATRFASVYAWNRKRINNCVADYSVLYNSTSFSTFKCYGVSPTKLNDLCFTNVYADSFVIRGDEVRQIAPGQTGKIADYNYKLPDDFTGCVIAWNSNTLDSKVGGNYTYLYRLFRKSNLKPFERDISTEIYQAGSTPCNGVEGFNCYFPLQSYGFQPTNGVGYQPYRVVVLSFELLHAPATVCGPKKSTNLVKNKSVNF

SEQ ID NO: 37 - protein, 223 aa, Artificial Sequence
  SARS-CoV-2 RBD S2004
RVQPTESIVRFPNITNLCPFGEVFNATRFASVYAWNRKRINNCVADYSVLYNSTSFSTFKCYGVSPTKLNDLCFTNVYADSFVIRGDEVRQIAPGQTGKIADYNYKLPDDFTGCVIAWNSNTLDSKVGGNYTYLYRLFRKSNLKPFERDISTEIYQAGSTPCNGVEGFNCYFPLQSYGFQPTNGVGYQPYRVVVLSFELLHAPATVCGPKKSTNLVKNKSVNF

SEQ ID NO: 38 - DNA, 931 bp, Artificial Sequence
  DNA insert
gtaatacgactcactataaggagacccaagctacatttgcttctgacacaactgtgttcactagcaacctcaaacagacaccgccaccatgttcgtgttcctggtgctgctgcccctggtgagcagcagagtgcagcccaccgagagcatcgtgcggttccccaacatcaccaacctgtgccccttcggcgaggtgttcaacgccaccagattcgccagcgtgtacgcctggaaccggaagcggatcagcaactgcgtggccgactacagcgtgctgtacaacagcgccagcttcagcaccttcaagtgctacggcgtgagccccaccaagctgaacgacctgtgcttcaccaacgtgtacgccgacagcttcgtgatcagaggcgacgaagtgcggcagatcgcccccggacagacaggcaacatcgccgactacaactacaagctgcccgacgacttcaccggctgcgtgatcgcctggaacagcaacaacctggacagcaaagtcggcggcaactacaactacctgtaccggctgttccggaagtccaacctgaagcccttcgagcgggacatcagcaccgagatctaccaggccggcagcaccccctgcaacggcgtgaaaggcttcaactgctacttcccactgcagagctacggcttccagcccacatacggcgtgggctaccagccctacagagtggtggtgctgagcttcgagctgctgcacgcccccgccacagtgtgcggccccaagaaaagcaccaacctggtcaagaacaaatgcgtgaacttctgagctcgctttcttgctgtccaatttctattaaaggttcctttgttccctaagtccaactactaaactgggggatattatgaagggccttgagcatctggattctgcctaataaaaaacatttattttcattgc

SEQ ID NO: 39 - DNA, 931 bp, Artificial Sequence
  DNA insert
gtaatacgactcactataaggagacccaagctacatttgcttctgacacaactgtgttcactagcaacctcaaacagacaccgccaccatgttcgtgttcctggtgctgctgcccctggtgagcagcagagtgcagcccaccgagagcatcgtgcggttccccaacatcaccaacctgtgccccttcggcgaggtgttcaacgccaccagattcgccagcgtgtacgcctggaaccggaagcggatcagcaactgcgtggccgactacagcgtgctgtacaacagcgccagcttcagcaccttcaagtgctacggcgtgagccccaccaagctgaacgacctgtgcttcaccaacgtgtacgccgacagcttcgtgatcagaggcgacgaagtgcggcagatcgcccccggacagacaggcaagatcgccgactacaactacaagctgcccgacgacttcaccggctgcgtgatcgcctggaacagcaacaacctggacagcaaagtcggcggcaactacaactacctgtaccggctgttccggaagtccaacctgaagcccttcgagcgggacatcagcaccgagatctaccaggccggcagcaccccctgcaacggcgtggaaggcttcaactgctacttcccactgcagagctacggcttccagcccacatacggcgtgggctaccagccctacagagtggtggtgctgagcttcgagctgctgcacgcccccgccacagtgtgcggccccaagaaaagcaccaacctggtcaagaacaaatgcgtgaacttctgagctcgctttcttgctgtccaatttctattaaaggttcctttgttccctaagtccaactactaaactgggggatattatgaagggccttgagcatctggattctgcctaataaaaaacatttattttcattgc

SEQ ID NO: 40 - DNA, 931 bp, Artificial Sequence
  DNA insert
gtaatacgactcactataaggagacccaagctacatttgcttctgacacaactgtgttcactagcaacctcaaacagacaccgccaccatgttcgtgttcctggtgctgctgcccctggtgagcagcagagtgcagcccaccgagagcatcgtgcggttccccaacatcaccaacctgtgccccttcggcgaggtgttcaacgccaccagattcgccagcgtgtacgcctggaaccggaagcggatcagcaactgcgtggccgactacagcgtgctgtacaacagcgccagcttcagcaccttcaagtgctacggcgtgagccccaccaagctgaacgacctgtgcttcaccaacgtgtacgccgacagcttcgtgatcagaggcgacgaagtgcggcagatcgcccccggacagacaggcacgatcgccgactacaactacaagctgcccgacgacttcaccggctgcgtgatcgcctggaacagcaacaacctggacagcaaagtcggcggcaactacaactacctgtaccggctgttccggaagtccaacctgaagcccttcgagcgggacatcagcaccgagatctaccaggccggcagcaccccctgcaacggcgtgaaaggcttcaactgctacttcccactgcagagctacggcttccagcccacatacggcgtgggctaccagccctacagagtggtggtgctgagcttcgagctgctgcacgcccccgccacagtgtgcggccccaagaaaagcaccaacctggtcaagaacaaatgcgtgaacttctgagctcgctttcttgctgtccaatttctattaaaggttcctttgttccctaagtccaactactaaactgggggatattatgaagggccttgagcatctggattctgcctaataaaaaacatttattttcattgc

SEQ ID NO: 41 - DNA, 931 bp, Artificial Sequence
  DNA insert
gtaatacgactcactataaggagacccaagctacatttgcttctgacacaactgtgttcactagcaacctcaaacagacaccgccaccatgttcgtgttcctggtgctgctgcccctggtgagcagcagagtgcagcccaccgagagcatcgtgcggttccccaacatcaccaacctgtgccccttcggcgaggtgttcaacgccaccagattcgccagcgtgtacgcctggaaccggaagcggatcagcaactgcgtggccgactacagcgtgctgtacaacagcgccagcttcagcaccttcaagtgctacggcgtgagccccaccaagctgaacgacctgtgcttcaccaacgtgtacgccgacagcttcgtgatcagaggcgacgaagtgcggcagatcgcccccggacagacaggcaagatcgccgactacaactacaagctgcccgacgacttcaccggctgcgtgatcgcctggaacagcaacaacctggacagcaaagtcggcggcaactacaactaccggtaccggctgttccggaagtccaacctgaagcccttcgagcgggacatcagcaccgagatctaccaggccggcagcaccccctgcaacggcgtggaaggcttcaactgctacttcccactgcagagctacggcttccagcccacaaacggcgtgggctaccagccctacagagtggtggtgctgagcttcgagctgctgcacgcccccgccacagtgtgcggccccaagaaaagcaccaacctggtcaagaacaaatgcgtgaacttctgagctcgctttcttgctgtccaatttctattaaaggttcctttgttccctaagtccaactactaaactgggggatattatgaagggccttgagcatctggattctgcctaataaaaaacatttattttcattgc

SEQ ID NO: 42 - DNA, 931 bp, Artificial Sequence
  DNA insert
gtaatacgactcactataaggagacccaagctacatttgcttctgacacaactgtgttcactagcaacctcaaacagacaccgccaccatgttcgtgttcctggtgctgctgcccctggtgagcagcagagtgcagcccaccgagagcatcgtgcggttccccaacatcaccaacctgtgccccttcggcgaggtgttcaacgccaccagattcgccagcgtgtacgcctggaaccggaagcggatcagcaactgcgtggccgactacagcgtgctgtacaacagcgccagcttcagcaccttcaagtgctacggcgtgagccccaccaagctgaacgacctgtgcttcaccaacgtgtacgccgacagcttcgtgatcagaggcgacgaagtgcggcagatcgcccccggacagacaggcaagatcgccgactacaactacaagctgcccgacgacttcaccggctgcgtgatcgcctggaacagcaacaacctggacagcaaagtcggcggcaactacaactaccggtaccggctgttccggaagtccaacctgaagcccttcgagcgggacatcagcaccgagatctaccaggccggcagcaccccctgcaacggcgtgcaaggcttcaactgctacttcccactgcagagctacggcttccagcccacaaacggcgtgggctaccagccctacagagtggtggtgctgagcttcgagctgctgcacgcccccgccacagtgtgcggccccaagaaaagcaccaacctggtcaagaacaaatgcgtgaacttctgagctcgctttcttgctgtccaatttctattaaaggttcctttgttccctaagtccaactactaaactgggggatattatgaagggccttgagcatctggattctgcctaataaaaaacatttattttcattgc

SEQ ID NO: 43 - DNA, 931 bp, Artificial Sequence
  DNA insert
gtaatacgactcactataaggagacccaagctacatttgcttctgacacaactgtgttcactagcaacctcaaacagacaccgccaccatgttcgtgttcctggtgctgctgcccctggtgagcagcagagtgcagcccaccgagagcatcgtgcggttccccaacatcaccaacctgtgccccttcggcgaggtgttcaacgccaccagattcgccagcgtgtacgcctggaaccggaagcggatcagcaactgcgtggccgactacagcgtgctgtacaacagcgccagcttcagcaccttcaagtgctacggcgtgagccccaccaagctgaacgacctgtgcttcaccaacgtgtacgccgacagcttcgtgatcagaggcgacgaagtgcggcagatcgcccccggacagacaggcaacatcgccgactacaactacaagctgcccgacgacttcaccggctgcgtgatcgcctggaacagcaacaacctggacagcaaagtcggcggcaactacaactacctgtaccggctgttccggaagtccaacctgaagcccttcgagcgggacatcagcaccgagatctaccaggccggcagcaccccctgcaacggcgtgaaaggcttcaactgctacttcccactgcagagctacggcttccagcccacatacggcgtgggctaccagccctacagagtggtggtgctgagcttcgagctgctgcacgcccccgccacagtgtgcggccccaagaaaagcaccaacctggtcaagaacaaaagcgtgaacttctgagctcgctttcttgctgtccaatttctattaaaggttcctttgttccctaagtccaactactaaactgggggatattatgaagggccttgagcatctggattctgcctaataaaaaacatttattttcattgc

SEQ ID NO: 44 - DNA, 931 bp, Artificial Sequence
  DNA insert
gtaatacgactcactataaggagacccaagctacatttgcttctgacacaactgtgttcactagcaacctcaaacagacaccgccaccatgttcgtgttcctggtgctgctgcccctggtgagcagcagagtgcagcccaccgagagcatcgtgcggttccccaacatcaccaacctgtgccccttcggcgaggtgttcaacgccaccagattcgccagcgtgtacgcctggaaccggaagcggatcagcaactgcgtggccgactacagcgtgctgtacaacagcgccagcttcagcaccttcaagtgctacggcgtgagccccaccaagctgaacgacctgtgcttcaccaacgtgtacgccgacagcttcgtgatcagaggcgacgaagtgcggcagatcgcccccggacagacaggcaagatcgccgactacaactacaagctgcccgacgacttcaccggctgcgtgatcgcctggaacagcaacaacctggacagcaaagtcggcggcaactacaactacctgtaccggctgttccggaagtccaacctgaagcccttcgagcgggacatcagcaccgagatctaccaggccggcagcaccccctgcaacggcgtggaaggcttcaactgctacttcccactgcagagctacggcttccagcccacatacggcgtgggctaccagccctacagagtggtggtgctgagcttcgagctgctgcacgcccccgccacagtgtgcggccccaagaaaagcaccaacctggtcaagaacaaaagcgtgaacttctgagctcgctttcttgctgtccaatttctattaaaggttcctttgttccctaagtccaactactaaactgggggatattatgaagggccttgagcatctggattctgcctaataaaaaacatttattttcattgc

SEQ ID NO: 45 - DNA, 931 bp, Artificial Sequence
  DNA insert
gtaatacgactcactataaggagacccaagctacatttgcttctgacacaactgtgttcactagcaacctcaaacagacaccgccaccatgttcgtgttcctggtgctgctgcccctggtgagcagcagagtgcagcccaccgagagcatcgtgcggttccccaacatcaccaacctgtgccccttcggcgaggtgttcaacgccaccagattcgccagcgtgtacgcctggaaccggaagcggatcagcaactgcgtggccgactacagcgtgctgtacaacagcgccagcttcagcaccttcaagtgctacggcgtgagccccaccaagctgaacgacctgtgcttcaccaacgtgtacgccgacagcttcgtgatcagaggcgacgaagtgcggcagatcgcccccggacagacaggcacgatcgccgactacaactacaagctgcccgacgacttcaccggctgcgtgatcgcctggaacagcaacaacctggacagcaaagtcggcggcaactacaactacctgtaccggctgttccggaagtccaacctgaagcccttcgagcgggacatcagcaccgagatctaccaggccggcagcaccccctgcaacggcgtgaaaggcttcaactgctacttcccactgcagagctacggcttccagcccacatacggcgtgggctaccagccctacagagtggtggtgctgagcttcgagctgctgcacgcccccgccacagtgtgcggccccaagaaaagcaccaacctggtcaagaacaaaagcgtgaacttctgagctcgctttcttgctgtccaatttctattaaaggttcctttgttccctaagtccaactactaaactgggggatattatgaagggccttgagcatctggattctgcctaataaaaaacatttattttcattgc

SEQ ID NO: 46 - DNA, 931 bp, Artificial Sequence
  DNA insert
gtaatacgactcactataaggagacccaagctacatttgcttctgacacaactgtgttcactagcaacctcaaacagacaccgccaccatgttcgtgttcctggtgctgctgcccctggtgagcagcagagtgcagcccaccgagagcatcgtgcggttccccaacatcaccaacctgtgccccttcggcgaggtgttcaacgccaccagattcgccagcgtgtacgcctggaaccggaagcggatcagcaactgcgtggccgactacagcgtgctgtacaacagcgccagcttcagcaccttcaagtgctacggcgtgagccccaccaagctgaacgacctgtgcttcaccaacgtgtacgccgacagcttcgtgatcagaggcgacgaagtgcggcagatcgcccccggacagacaggcaagatcgccgactacaactacaagctgcccgacgacttcaccggctgcgtgatcgcctggaacagcaacaacctggacagcaaagtcggcggcaactacaactaccggtaccggctgttccggaagtccaacctgaagcccttcgagcgggacatcagcaccgagatctaccaggccggcagcaccccctgcaacggcgtggaaggcttcaactgctacttcccactgcagagctacggcttccagcccacaaacggcgtgggctaccagccctacagagtggtggtgctgagcttcgagctgctgcacgcccccgccacagtgtgcggccccaagaaaagcaccaacctggtcaagaacaaaagcgtgaacttctgagctcgctttcttgctgtccaatttctattaaaggttcctttgttccctaagtccaactactaaactgggggatattatgaagggccttgagcatctggattctgcctaataaaaaacatttattttcattgc

SEQ ID NO: 47 - DNA, 931 bp, Artificial Sequence
  DNA insert
gtaatacgactcactataaggagacccaagctacatttgcttctgacacaactgtgttcactagcaacctcaaacagacaccgccaccatgttcgtgttcctggtgctgctgcccctggtgagcagcagagtgcagcccaccgagagcatcgtgcggttccccaacatcaccaacctgtgccccttcggcgaggtgttcaacgccaccagattcgccagcgtgtacgcctggaaccggaagcggatcagcaactgcgtggccgactacagcgtgctgtacaacagcgccagcttcagcaccttcaagtgctacggcgtgagccccaccaagctgaacgacctgtgcttcaccaacgtgtacgccgacagcttcgtgatcagaggcgacgaagtgcggcagatcgcccccggacagacaggcaagatcgccgactacaactacaagctgcccgacgacttcaccggctgcgtgatcgcctggaacagcaacaacctggacagcaaagtcggcggcaactacaactaccggtaccggctgttccggaagtccaacctgaagcccttcgagcgggacatcagcaccgagatctaccaggccggcagcaccccctgcaacggcgtgcaaggcttcaactgctacttcccactgcagagctacggcttccagcccacaaacggcgtgggctaccagccctacagagtggtggtgctgagcttcgagctgctgcacgcccccgccacagtgtgcggccccaagaaaagcaccaacctggtcaagaacaaaagcgtgaacttctgagctcgctttcttgctgtccaatttctattaaaggttcctttgttccctaagtccaactactaaactgggggatattatgaagggccttgagcatctggattctgcctaataaaaaacatttattttcattgc

SEQ ID NO: 48 - DNA, 931 bp, Artificial Sequence
  DNA insert
gtaatacgactcactataaggagacccaagctacatttgcttctgacacaactgtgttcactagcaacctcaaacagacaccgccaccatgttcgtgttcctggtgctgctgcccctggtgagcagcagagtgcagcccaccgagagcatcgtgcggttccccaacatcaccaacctgtgccccttcggcgaggtgttcaacgccaccagattcgccagcgtgtacgcctggaaccggaagcggatcagcaactgcgtggccgactacagcgtgctgtacaacagcgccagcttcagcaccttcaagtgctacggcgtgagccccaccaagctgaacgacctgtgcttcaccaacgtgtacgccgacagcttcgtgatcagaggcgacgaagtgcggcagatcgcccccggacagacaggcaagatcgccgactacaactacaagctgcccgacgacttcaccggctgcgtgatcgcctggaacagcaagaacctggacagcaaagtcggcggcaactacaactaccggtaccggctgttccggaagtccaacctgaagcccttcgagcgggacatcagcaccgagatctaccaggtcggcagcaccccctgcaacggcgcggaaggcttcaactgctacttcccactgcagagctacggcttccagcccacaaacggcgtgggctaccagccctacagagtggtggtgctgagcttcgagctgctgcacgcccccgccacagtgtgcggccccaagaaaagcaccaacctggtcaagaacaaatgcgtgaacttctgagctcgctttcttgctgtccaatttctattaaaggttcctttgttccctaagtccaactactaaactgggggatattatgaagggccttgagcatctggattctgcctaataaaaaacatttattttcattgc

SEQ ID NO: 49 - DNA, 931 bp, Artificial Sequence
  DNA insert
gtaatacgactcactataaggagacccaagctacatttgcttctgacacaactgtgttcactagcaacctcaaacagacaccgccaccatgttcgtgttcctggtgctgctgcccctggtgagcagcagagtgcagcccaccgagagcatcgtgcggttccccaacatcaccaacctgtgccccttcggcgaggtgttcaacgccaccagattcgccagcgtgtacgcctggaaccggaagcggatcagcaactgcgtggccgactacagcgtgctgtacaacagcgccagcttcagcaccttcaagtgctacggcgtgagccccaccaagctgaacgacctgtgcttcaccaacgtgtacgccgacagcttcgtgatcagaggcgacgaagtgcggcagatcgcccccggacagacaggcaagatcgccgactacaactacaagctgcccgacgacttcaccggctgcgtgatcgcctggaacagcaacaacctggacagcaaagtcggcggcaactacaactacctgtaccggctgttccggaagtccaacctgaagcccttcgagcgggacatcagcaccgagatctaccaggccggcagaaccccctgcaacggcgtggaaggcttcaactgctacctcccactgcagagctacggcttccagcccacaaacggcgtgggctaccagccctacagagtggtggtgctgagcttcgagctgctgcacgcccccgccacagtgtgcggccccaagaaaagcaccaacctggtcaagaacaaatgcgtgaacttctgagctcgctttcttgctgtccaatttctattaaaggttcctttgttccctaagtccaactactaaactgggggatattatgaagggccttgagcatctggattctgcctaataaaaaacatttattttcattgc

SEQ ID NO: 50 - DNA, 931 bp, Artificial Sequence
  DNA insert
gtaatacgactcactataaggagacccaagctacatttgcttctgacacaactgtgttcactagcaacctcaaacagacaccgccaccatgttcgtgttcctggtgctgctgcccctggtgagcagcagagtgcagcccaccgagagcatcgtgcggttccccaacatcaccaacctgtgccccttcggcgaggtgttcaacgccaccagattcgccagcgtgtacgcctggaaccggaagcggatcagcaactgcgtggccgactacagcgtgctgtacaacagcgccagcttcagcaccttcaagtgctacggcgtgagccccaccaagctgaacgacctgtgcttcaccaacgtgtacgccgacagcttcgtgatcagaggcgacgaagtgcggcagatcgcccccggacagacaggcaacatcgccgactacaactacaagctgcccgacgacttcaccggctgcgtgatcgcctggaacagcaacaacctggacagcaaagtcggcggcaactacaactacctgtaccggctgttccggaagtccaacctgaagcccttcgagcgggacatcagcaccgagatctaccaggccggcagaaccccctgcaacggcgtgaaaggcttcaactgctacttcccactgcagagctacggcttccagcccacatacggcgtgggctaccagccctacagagtggtggtgctgagcttcgagctgctgcacgcccccgccacagtgtgcggccccaagaaaagcaccaacctggtcaagaacaaatgcgtgaacttctgagctcgctttcttgctgtccaatttctattaaaggttcctttgttccctaagtccaactactaaactgggggatattatgaagggccttgagcatctggattctgcctaataaaaaacatttattttcattgc

SEQ ID NO: 51 - DNA, 931 bp, Artificial Sequence
  DNA insert
gtaatacgactcactataaggagacccaagctacatttgcttctgacacaactgtgttcactagcaacctcaaacagacaccgccaccatgttcgtgttcctggtgctgctgcccctggtgagcagcagagtgcagcccaccgagagcatcgtgcggttccccaacatcaccaacctgtgccccttcggcgaggtgttcaacgccaccagattcgccagcgtgtacgcctggaaccggaagcggatcagcaactgcgtggccgactacagcgtgctgtacaacagcgccagcttcagcaccttcaagtgctacggcgtgagccccaccaagctgaacgacctgtgcttcaccaacgtgtacgccgacagcttcgtgatcagaggcgacgaagtgcggcagatcgcccccggacagacaggcaagatcgccgactacaactacaagctgcccgacgacttcaccggctgcgtgatcgcctggaacagcaacaacctggacagcaaagtcggcggcaactacaactacctgtaccggctgttccggaagtccaacctgaagcccttcgagcgggacatcagcaccgagatctaccaggccggcagcaccccctgcaacggcgtggaaggcagcaactgctacctcccactgcagagctacggcttccagcccacaaacggcgtgggctaccagccctacagagtggtggtgctgagcttcgagctgctgcacgcccccgccacagtgtgcggccccaagaaaagcaccaacctggtcaagaacaaatgcgtgaacttctgagctcgctttcttgctgtccaatttctattaaaggttcctttgttccctaagtccaactactaaactgggggatattatgaagggccttgagcatctggattctgcctaataaaaaacatttattttcattgc

SEQ ID NO: 52 - DNA, 1031 bp, Artificial Sequence
  template DNA
gtaatacgactcactataaggagacccaagctacatttgcttctgacacaactgtgttcactagcaacctcaaacagacaccgccaccatgttcgtgttcctggtgctgctgcccctggtgagcagcagagtgcagcccaccgagagcatcgtgcggttccccaacatcaccaacctgtgccccttcggcgaggtgttcaacgccaccagattcgccagcgtgtacgcctggaaccggaagcggatcagcaactgcgtggccgactacagcgtgctgtacaacagcgccagcttcagcaccttcaagtgctacggcgtgagccccaccaagctgaacgacctgtgcttcaccaacgtgtacgccgacagcttcgtgatcagaggcgacgaagtgcggcagatcgcccccggacagacaggcaacatcgccgactacaactacaagctgcccgacgacttcaccggctgcgtgatcgcctggaacagcaacaacctggacagcaaagtcggcggcaactacaactacctgtaccggctgttccggaagtccaacctgaagcccttcgagcgggacatcagcaccgagatctaccaggccggcagcaccccctgcaacggcgtgaaaggcttcaactgctacttcccactgcagagctacggcttccagcccacatacggcgtgggctaccagccctacagagtggtggtgctgagcttcgagctgctgcacgcccccgccacagtgtgcggccccaagaaaagcaccaacctggtcaagaacaaatgcgtgaacttctgagctcgctttcttgctgtccaatttctattaaaggttcctttgttccctaagtccaactactaaactgggggatattatgaagggccttgagcatctggattctgcctaataaaaaacatttattttcattgcaaaaaaaaaaaaaaaaaaaaaaaaaaaaaaaaaaaaaaaaaaaaaaaaaaaaaaaaaaaaaaaaaaaaaaaaaaaaaaaaaaaaaaaaaaaaaaaaaaaa

SEQ ID NO: 53 - DNA, 1031 bp, Artificial Sequence
  template DNA
gtaatacgactcactataaggagacccaagctacatttgcttctgacacaactgtgttcactagcaacctcaaacagacaccgccaccatgttcgtgttcctggtgctgctgcccctggtgagcagcagagtgcagcccaccgagagcatcgtgcggttccccaacatcaccaacctgtgccccttcggcgaggtgttcaacgccaccagattcgccagcgtgtacgcctggaaccggaagcggatcagcaactgcgtggccgactacagcgtgctgtacaacagcgccagcttcagcaccttcaagtgctacggcgtgagccccaccaagctgaacgacctgtgcttcaccaacgtgtacgccgacagcttcgtgatcagaggcgacgaagtgcggcagatcgcccccggacagacaggcaagatcgccgactacaactacaagctgcccgacgacttcaccggctgcgtgatcgcctggaacagcaacaacctggacagcaaagtcggcggcaactacaactacctgtaccggctgttccggaagtccaacctgaagcccttcgagcgggacatcagcaccgagatctaccaggccggcagcaccccctgcaacggcgtggaaggcttcaactgctacttcccactgcagagctacggcttccagcccacatacggcgtgggctaccagccctacagagtggtggtgctgagcttcgagctgctgcacgcccccgccacagtgtgcggccccaagaaaagcaccaacctggtcaagaacaaatgcgtgaacttctgagctcgctttcttgctgtccaatttctattaaaggttcctttgttccctaagtccaactactaaactgggggatattatgaagggccttgagcatctggattctgcctaataaaaaacatttattttcattgcaaaaaaaaaaaaaaaaaaaaaaaaaaaaaaaaaaaaaaaaaaaaaaaaaaaaaaaaaaaaaaaaaaaaaaaaaaaaaaaaaaaaaaaaaaaaaaaaaaaa

SEQ ID NO: 54 - DNA, 1031 bp, Artificial Sequence
  template DNA
gtaatacgactcactataaggagacccaagctacatttgcttctgacacaactgtgttcactagcaacctcaaacagacaccgccaccatgttcgtgttcctggtgctgctgcccctggtgagcagcagagtgcagcccaccgagagcatcgtgcggttccccaacatcaccaacctgtgccccttcggcgaggtgttcaacgccaccagattcgccagcgtgtacgcctggaaccggaagcggatcagcaactgcgtggccgactacagcgtgctgtacaacagcgccagcttcagcaccttcaagtgctacggcgtgagccccaccaagctgaacgacctgtgcttcaccaacgtgtacgccgacagcttcgtgatcagaggcgacgaagtgcggcagatcgcccccggacagacaggcacgatcgccgactacaactacaagctgcccgacgacttcaccggctgcgtgatcgcctggaacagcaacaacctggacagcaaagtcggcggcaactacaactacctgtaccggctgttccggaagtccaacctgaagcccttcgagcgggacatcagcaccgagatctaccaggccggcagcaccccctgcaacggcgtgaaaggcttcaactgctacttcccactgcagagctacggcttccagcccacatacggcgtgggctaccagccctacagagtggtggtgctgagcttcgagctgctgcacgcccccgccacagtgtgcggccccaagaaaagcaccaacctggtcaagaacaaatgcgtgaacttctgagctcgctttcttgctgtccaatttctattaaaggttcctttgttccctaagtccaactactaaactgggggatattatgaagggccttgagcatctggattctgcctaataaaaaacatttattttcattgcaaaaaaaaaaaaaaaaaaaaaaaaaaaaaaaaaaaaaaaaaaaaaaaaaaaaaaaaaaaaaaaaaaaaaaaaaaaaaaaaaaaaaaaaaaaaaaaaaaaa

SEQ ID NO: 55 - DNA, 1031 bp, Artificial Sequence
  template DNA
gtaatacgactcactataaggagacccaagctacatttgcttctgacacaactgtgttcactagcaacctcaaacagacaccgccaccatgttcgtgttcctggtgctgctgcccctggtgagcagcagagtgcagcccaccgagagcatcgtgcggttccccaacatcaccaacctgtgccccttcggcgaggtgttcaacgccaccagattcgccagcgtgtacgcctggaaccggaagcggatcagcaactgcgtggccgactacagcgtgctgtacaacagcgccagcttcagcaccttcaagtgctacggcgtgagccccaccaagctgaacgacctgtgcttcaccaacgtgtacgccgacagcttcgtgatcagaggcgacgaagtgcggcagatcgcccccggacagacaggcaagatcgccgactacaactacaagctgcccgacgacttcaccggctgcgtgatcgcctggaacagcaacaacctggacagcaaagtcggcggcaactacaactaccggtaccggctgttccggaagtccaacctgaagcccttcgagcgggacatcagcaccgagatctaccaggccggcagcaccccctgcaacggcgtggaaggcttcaactgctacttcccactgcagagctacggcttccagcccacaaacggcgtgggctaccagccctacagagtggtggtgctgagcttcgagctgctgcacgcccccgccacagtgtgcggccccaagaaaagcaccaacctggtcaagaacaaatgcgtgaacttctgagctcgctttcttgctgtccaatttctattaaaggttcctttgttccctaagtccaactactaaactgggggatattatgaagggccttgagcatctggattctgcctaataaaaaacatttattttcattgcaaaaaaaaaaaaaaaaaaaaaaaaaaaaaaaaaaaaaaaaaaaaaaaaaaaaaaaaaaaaaaaaaaaaaaaaaaaaaaaaaaaaaaaaaaaaaaaaaaaa

SEQ ID NO: 56 - DNA, 1031 bp, Artificial Sequence
  template DNA
gtaatacgactcactataaggagacccaagctacatttgcttctgacacaactgtgttcactagcaacctcaaacagacaccgccaccatgttcgtgttcctggtgctgctgcccctggtgagcagcagagtgcagcccaccgagagcatcgtgcggttccccaacatcaccaacctgtgccccttcggcgaggtgttcaacgccaccagattcgccagcgtgtacgcctggaaccggaagcggatcagcaactgcgtggccgactacagcgtgctgtacaacagcgccagcttcagcaccttcaagtgctacggcgtgagccccaccaagctgaacgacctgtgcttcaccaacgtgtacgccgacagcttcgtgatcagaggcgacgaagtgcggcagatcgcccccggacagacaggcaagatcgccgactacaactacaagctgcccgacgacttcaccggctgcgtgatcgcctggaacagcaacaacctggacagcaaagtcggcggcaactacaactaccggtaccggctgttccggaagtccaacctgaagcccttcgagcgggacatcagcaccgagatctaccaggccggcagcaccccctgcaacggcgtgcaaggcttcaactgctacttcccactgcagagctacggcttccagcccacaaacggcgtgggctaccagccctacagagtggtggtgctgagcttcgagctgctgcacgcccccgccacagtgtgcggccccaagaaaagcaccaacctggtcaagaacaaatgcgtgaacttctgagctcgctttcttgctgtccaatttctattaaaggttcctttgttccctaagtccaactactaaactgggggatattatgaagggccttgagcatctggattctgcctaataaaaaacatttattttcattgcaaaaaaaaaaaaaaaaaaaaaaaaaaaaaaaaaaaaaaaaaaaaaaaaaaaaaaaaaaaaaaaaaaaaaaaaaaaaaaaaaaaaaaaaaaaaaaaaaaaa

SEQ ID NO: 57 - DNA, 1031 bp, Artificial Sequence
  template DNA
gtaatacgactcactataaggagacccaagctacatttgcttctgacacaactgtgttcactagcaacctcaaacagacaccgccaccatgttcgtgttcctggtgctgctgcccctggtgagcagcagagtgcagcccaccgagagcatcgtgcggttccccaacatcaccaacctgtgccccttcggcgaggtgttcaacgccaccagattcgccagcgtgtacgcctggaaccggaagcggatcagcaactgcgtggccgactacagcgtgctgtacaacagcgccagcttcagcaccttcaagtgctacggcgtgagccccaccaagctgaacgacctgtgcttcaccaacgtgtacgccgacagcttcgtgatcagaggcgacgaagtgcggcagatcgcccccggacagacaggcaacatcgccgactacaactacaagctgcccgacgacttcaccggctgcgtgatcgcctggaacagcaacaacctggacagcaaagtcggcggcaactacaactacctgtaccggctgttccggaagtccaacctgaagcccttcgagcgggacatcagcaccgagatctaccaggccggcagcaccccctgcaacggcgtgaaaggcttcaactgctacttcccactgcagagctacggcttccagcccacatacggcgtgggctaccagccctacagagtggtggtgctgagcttcgagctgctgcacgcccccgccacagtgtgcggccccaagaaaagcaccaacctggtcaagaacaaaagcgtgaacttctgagctcgctttcttgctgtccaatttctattaaaggttcctttgttccctaagtccaactactaaactgggggatattatgaagggccttgagcatctggattctgcctaataaaaaacatttattttcattgcaaaaaaaaaaaaaaaaaaaaaaaaaaaaaaaaaaaaaaaaaaaaaaaaaaaaaaaaaaaaaaaaaaaaaaaaaaaaaaaaaaaaaaaaaaaaaaaaaaaa

SEQ ID NO: 58 - DNA, 1031 bp, Artificial Sequence
  template DNA
gtaatacgactcactataaggagacccaagctacatttgcttctgacacaactgtgttcactagcaacctcaaacagacaccgccaccatgttcgtgttcctggtgctgctgcccctggtgagcagcagagtgcagcccaccgagagcatcgtgcggttccccaacatcaccaacctgtgccccttcggcgaggtgttcaacgccaccagattcgccagcgtgtacgcctggaaccggaagcggatcagcaactgcgtggccgactacagcgtgctgtacaacagcgccagcttcagcaccttcaagtgctacggcgtgagccccaccaagctgaacgacctgtgcttcaccaacgtgtacgccgacagcttcgtgatcagaggcgacgaagtgcggcagatcgcccccggacagacaggcaagatcgccgactacaactacaagctgcccgacgacttcaccggctgcgtgatcgcctggaacagcaacaacctggacagcaaagtcggcggcaactacaactacctgtaccggctgttccggaagtccaacctgaagcccttcgagcgggacatcagcaccgagatctaccaggccggcagcaccccctgcaacggcgtggaaggcttcaactgctacttcccactgcagagctacggcttccagcccacatacggcgtgggctaccagccctacagagtggtggtgctgagcttcgagctgctgcacgcccccgccacagtgtgcggccccaagaaaagcaccaacctggtcaagaacaaaagcgtgaacttctgagctcgctttcttgctgtccaatttctattaaaggttcctttgttccctaagtccaactactaaactgggggatattatgaagggccttgagcatctggattctgcctaataaaaaacatttattttcattgcaaaaaaaaaaaaaaaaaaaaaaaaaaaaaaaaaaaaaaaaaaaaaaaaaaaaaaaaaaaaaaaaaaaaaaaaaaaaaaaaaaaaaaaaaaaaaaaaaaaa

SEQ ID NO: 59 - DNA, 1031 bp, Artificial Sequence
  template DNA
gtaatacgactcactataaggagacccaagctacatttgcttctgacacaactgtgttcactagcaacctcaaacagacaccgccaccatgttcgtgttcctggtgctgctgcccctggtgagcagcagagtgcagcccaccgagagcatcgtgcggttccccaacatcaccaacctgtgccccttcggcgaggtgttcaacgccaccagattcgccagcgtgtacgcctggaaccggaagcggatcagcaactgcgtggccgactacagcgtgctgtacaacagcgccagcttcagcaccttcaagtgctacggcgtgagccccaccaagctgaacgacctgtgcttcaccaacgtgtacgccgacagcttcgtgatcagaggcgacgaagtgcggcagatcgcccccggacagacaggcacgatcgccgactacaactacaagctgcccgacgacttcaccggctgcgtgatcgcctggaacagcaacaacctggacagcaaagtcggcggcaactacaactacctgtaccggctgttccggaagtccaacctgaagcccttcgagcgggacatcagcaccgagatctaccaggccggcagcaccccctgcaacggcgtgaaaggcttcaactgctacttcccactgcagagctacggcttccagcccacatacggcgtgggctaccagccctacagagtggtggtgctgagcttcgagctgctgcacgcccccgccacagtgtgcggccccaagaaaagcaccaacctggtcaagaacaaaagcgtgaacttctgagctcgctttcttgctgtccaatttctattaaaggttcctttgttccctaagtccaactactaaactgggggatattatgaagggccttgagcatctggattctgcctaataaaaaacatttattttcattgcaaaaaaaaaaaaaaaaaaaaaaaaaaaaaaaaaaaaaaaaaaaaaaaaaaaaaaaaaaaaaaaaaaaaaaaaaaaaaaaaaaaaaaaaaaaaaaaaaaaa

SEQ ID NO: 60 - DNA, 1031 bp, Artificial Sequence
  template DNA
gtaatacgactcactataaggagacccaagctacatttgcttctgacacaactgtgttcactagcaacctcaaacagacaccgccaccatgttcgtgttcctggtgctgctgcccctggtgagcagcagagtgcagcccaccgagagcatcgtgcggttccccaacatcaccaacctgtgccccttcggcgaggtgttcaacgccaccagattcgccagcgtgtacgcctggaaccggaagcggatcagcaactgcgtggccgactacagcgtgctgtacaacagcgccagcttcagcaccttcaagtgctacggcgtgagccccaccaagctgaacgacctgtgcttcaccaacgtgtacgccgacagcttcgtgatcagaggcgacgaagtgcggcagatcgcccccggacagacaggcaagatcgccgactacaactacaagctgcccgacgacttcaccggctgcgtgatcgcctggaacagcaacaacctggacagcaaagtcggcggcaactacaactaccggtaccggctgttccggaagtccaacctgaagcccttcgagcgggacatcagcaccgagatctaccaggccggcagcaccccctgcaacggcgtggaaggcttcaactgctacttcccactgcagagctacggcttccagcccacaaacggcgtgggctaccagccctacagagtggtggtgctgagcttcgagctgctgcacgcccccgccacagtgtgcggccccaagaaaagcaccaacctggtcaagaacaaaagcgtgaacttctgagctcgctttcttgctgtccaatttctattaaaggttcctttgttccctaagtccaactactaaactgggggatattatgaagggccttgagcatctggattctgcctaataaaaaacatttattttcattgcaaaaaaaaaaaaaaaaaaaaaaaaaaaaaaaaaaaaaaaaaaaaaaaaaaaaaaaaaaaaaaaaaaaaaaaaaaaaaaaaaaaaaaaaaaaaaaaaaaaa

SEQ ID NO: 61 - DNA, 1031 bp, Artificial Sequence
  template DNA
gtaatacgactcactataaggagacccaagctacatttgcttctgacacaactgtgttcactagcaacctcaaacagacaccgccaccatgttcgtgttcctggtgctgctgcccctggtgagcagcagagtgcagcccaccgagagcatcgtgcggttccccaacatcaccaacctgtgccccttcggcgaggtgttcaacgccaccagattcgccagcgtgtacgcctggaaccggaagcggatcagcaactgcgtggccgactacagcgtgctgtacaacagcgccagcttcagcaccttcaagtgctacggcgtgagccccaccaagctgaacgacctgtgcttcaccaacgtgtacgccgacagcttcgtgatcagaggcgacgaagtgcggcagatcgcccccggacagacaggcaagatcgccgactacaactacaagctgcccgacgacttcaccggctgcgtgatcgcctggaacagcaacaacctggacagcaaagtcggcggcaactacaactaccggtaccggctgttccggaagtccaacctgaagcccttcgagcgggacatcagcaccgagatctaccaggccggcagcaccccctgcaacggcgtgcaaggcttcaactgctacttcccactgcagagctacggcttccagcccacaaacggcgtgggctaccagccctacagagtggtggtgctgagcttcgagctgctgcacgcccccgccacagtgtgcggccccaagaaaagcaccaacctggtcaagaacaaaagcgtgaacttctgagctcgctttcttgctgtccaatttctattaaaggttcctttgttccctaagtccaactactaaactgggggatattatgaagggccttgagcatctggattctgcctaataaaaaacatttattttcattgcaaaaaaaaaaaaaaaaaaaaaaaaaaaaaaaaaaaaaaaaaaaaaaaaaaaaaaaaaaaaaaaaaaaaaaaaaaaaaaaaaaaaaaaaaaaaaaaaaaaa

SEQ ID NO: 62 - DNA, 1031 bp, Artificial Sequence
  template DNA
gtaatacgactcactataaggagacccaagctacatttgcttctgacacaactgtgttcactagcaacctcaaacagacaccgccaccatgttcgtgttcctggtgctgctgcccctggtgagcagcagagtgcagcccaccgagagcatcgtgcggttccccaacatcaccaacctgtgccccttcggcgaggtgttcaacgccaccagattcgccagcgtgtacgcctggaaccggaagcggatcagcaactgcgtggccgactacagcgtgctgtacaacagcgccagcttcagcaccttcaagtgctacggcgtgagccccaccaagctgaacgacctgtgcttcaccaacgtgtacgccgacagcttcgtgatcagaggcgacgaagtgcggcagatcgcccccggacagacaggcaagatcgccgactacaactacaagctgcccgacgacttcaccggctgcgtgatcgcctggaacagcaagaacctggacagcaaagtcggcggcaactacaactaccggtaccggctgttccggaagtccaacctgaagcccttcgagcgggacatcagcaccgagatctaccaggtcggcagcaccccctgcaacggcgcggaaggcttcaactgctacttcccactgcagagctacggcttccagcccacaaacggcgtgggctaccagccctacagagtggtggtgctgagcttcgagctgctgcacgcccccgccacagtgtgcggccccaagaaaagcaccaacctggtcaagaacaaatgcgtgaacttctgagctcgctttcttgctgtccaatttctattaaaggttcctttgttccctaagtccaactactaaactgggggatattatgaagggccttgagcatctggattctgcctaataaaaaacatttattttcattgcaaaaaaaaaaaaaaaaaaaaaaaaaaaaaaaaaaaaaaaaaaaaaaaaaaaaaaaaaaaaaaaaaaaaaaaaaaaaaaaaaaaaaaaaaaaaaaaaaaaa

SEQ ID NO: 63 - DNA, 1031 bp, Artificial Sequence
  template DNA
gtaatacgactcactataaggagacccaagctacatttgcttctgacacaactgtgttcactagcaacctcaaacagacaccgccaccatgttcgtgttcctggtgctgctgcccctggtgagcagcagagtgcagcccaccgagagcatcgtgcggttccccaacatcaccaacctgtgccccttcggcgaggtgttcaacgccaccagattcgccagcgtgtacgcctggaaccggaagcggatcagcaactgcgtggccgactacagcgtgctgtacaacagcgccagcttcagcaccttcaagtgctacggcgtgagccccaccaagctgaacgacctgtgcttcaccaacgtgtacgccgacagcttcgtgatcagaggcgacgaagtgcggcagatcgcccccggacagacaggcaagatcgccgactacaactacaagctgcccgacgacttcaccggctgcgtgatcgcctggaacagcaacaacctggacagcaaagtcggcggcaactacaactacctgtaccggctgttccggaagtccaacctgaagcccttcgagcgggacatcagcaccgagatctaccaggccggcagaaccccctgcaacggcgtggaaggcttcaactgctacctcccactgcagagctacggcttccagcccacaaacggcgtgggctaccagccctacagagtggtggtgctgagcttcgagctgctgcacgcccccgccacagtgtgcggccccaagaaaagcaccaacctggtcaagaacaaatgcgtgaacttctgagctcgctttcttgctgtccaatttctattaaaggttcctttgttccctaagtccaactactaaactgggggatattatgaagggccttgagcatctggattctgcctaataaaaaacatttattttcattgcaaaaaaaaaaaaaaaaaaaaaaaaaaaaaaaaaaaaaaaaaaaaaaaaaaaaaaaaaaaaaaaaaaaaaaaaaaaaaaaaaaaaaaaaaaaaaaaaaaaa

SEQ ID NO: 64 - DNA, 1031 bp, Artificial Sequence
  template DNA
gtaatacgactcactataaggagacccaagctacatttgcttctgacacaactgtgttcactagcaacctcaaacagacaccgccaccatgttcgtgttcctggtgctgctgcccctggtgagcagcagagtgcagcccaccgagagcatcgtgcggttccccaacatcaccaacctgtgccccttcggcgaggtgttcaacgccaccagattcgccagcgtgtacgcctggaaccggaagcggatcagcaactgcgtggccgactacagcgtgctgtacaacagcgccagcttcagcaccttcaagtgctacggcgtgagccccaccaagctgaacgacctgtgcttcaccaacgtgtacgccgacagcttcgtgatcagaggcgacgaagtgcggcagatcgcccccggacagacaggcaacatcgccgactacaactacaagctgcccgacgacttcaccggctgcgtgatcgcctggaacagcaacaacctggacagcaaagtcggcggcaactacaactacctgtaccggctgttccggaagtccaacctgaagcccttcgagcgggacatcagcaccgagatctaccaggccggcagaaccccctgcaacggcgtgaaaggcttcaactgctacttcccactgcagagctacggcttccagcccacatacggcgtgggctaccagccctacagagtggtggtgctgagcttcgagctgctgcacgcccccgccacagtgtgcggccccaagaaaagcaccaacctggtcaagaacaaatgcgtgaacttctgagctcgctttcttgctgtccaatttctattaaaggttcctttgttccctaagtccaactactaaactgggggatattatgaagggccttgagcatctggattctgcctaataaaaaacatttattttcattgcaaaaaaaaaaaaaaaaaaaaaaaaaaaaaaaaaaaaaaaaaaaaaaaaaaaaaaaaaaaaaaaaaaaaaaaaaaaaaaaaaaaaaaaaaaaaaaaaaaaa

SEQ ID NO: 65 - DNA, 1031 bp, Artificial Sequence
  template DNA
gtaatacgactcactataaggagacccaagctacatttgcttctgacacaactgtgttcactagcaacctcaaacagacaccgccaccatgttcgtgttcctggtgctgctgcccctggtgagcagcagagtgcagcccaccgagagcatcgtgcggttccccaacatcaccaacctgtgccccttcggcgaggtgttcaacgccaccagattcgccagcgtgtacgcctggaaccggaagcggatcagcaactgcgtggccgactacagcgtgctgtacaacagcgccagcttcagcaccttcaagtgctacggcgtgagccccaccaagctgaacgacctgtgcttcaccaacgtgtacgccgacagcttcgtgatcagaggcgacgaagtgcggcagatcgcccccggacagacaggcaagatcgccgactacaactacaagctgcccgacgacttcaccggctgcgtgatcgcctggaacagcaacaacctggacagcaaagtcggcggcaactacaactacctgtaccggctgttccggaagtccaacctgaagcccttcgagcgggacatcagcaccgagatctaccaggccggcagcaccccctgcaacggcgtggaaggcagcaactgctacctcccactgcagagctacggcttccagcccacaaacggcgtgggctaccagccctacagagtggtggtgctgagcttcgagctgctgcacgcccccgccacagtgtgcggccccaagaaaagcaccaacctggtcaagaacaaatgcgtgaacttctgagctcgctttcttgctgtccaatttctattaaaggttcctttgttccctaagtccaactactaaactgggggatattatgaagggccttgagcatctggattctgcctaataaaaaacatttattttcattgcaaaaaaaaaaaaaaaaaaaaaaaaaaaaaaaaaaaaaaaaaaaaaaaaaaaaaaaaaaaaaaaaaaaaaaaaaaaaaaaaaaaaaaaaaaaaaaaaaaaa

SEQ ID NO: 66 - RNA, 1013 nt, Artificial Sequence
  SARS-CoV-2 variant RBD mRNA (South African variant)
aggagacccaagcuacauuugcuucugacacaacuguguucacuagcaaccucaaacagacaccgccaccauguucguguuccuggugcugcugccccuggugagcagcagagugcagcccaccgagagcaucgugcgguuccccaacaucaccaaccugugccccuucggcgagguguucaacgccaccagauucgccagcguguacgccuggaaccggaagcggaucagcaacugcguggccgacuacagcgugcuguacaacagcgccagcuucagcaccuucaagugcuacggcgugagccccaccaagcugaacgaccugugcuucaccaacguguacgccgacagcuucgugaucagaggcgacgaagugcggcagaucgcccccggacagacaggcaacaucgccgacuacaacuacaagcugcccgacgacuucaccggcugcgugaucgccuggaacagcaacaaccuggacagcaaagucggcggcaacuacaacuaccuguaccggcuguuccggaaguccaaccugaagcccuucgagcgggacaucagcaccgagaucuaccaggccggcagcacccccugcaacggcgugaaaggcuucaacugcuacuucccacugcagagcuacggcuuccagcccacauacggcgugggcuaccagcccuacagagugguggugcugagcuucgagcugcugcacgcccccgccacagugugcggccccaagaaaagcaccaaccuggucaagaacaaaugcgugaacuucugagcucgcuuucuugcuguccaauuucuauuaaagguuccuuuguucccuaaguccaacuacuaaacugggggauauuaugaagggccuugagcaucuggauucugccuaauaaaaaacauuuauuuucauugcaaaaaaaaaaaaaaaaaaaaaaaaaaaaaaaaaaaaaaaaaaaaaaaaaaaaaaaaaaaaaaaaaaaaaaaaaaaaaaaaaaaaaaaaaaaaaaaaaaaa

SEQ ID NO: 67 - RNA, 1013 nt, Artificial Sequence
  SARS-CoV-2 variant RBD mRNA (UK variant)
aggagacccaagcuacauuugcuucugacacaacuguguucacuagcaaccucaaacagacaccgccaccauguucguguuccuggugcugcugccccuggugagcagcagagugcagcccaccgagagcaucgugcgguuccccaacaucaccaaccugugccccuucggcgagguguucaacgccaccagauucgccagcguguacgccuggaaccggaagcggaucagcaacugcguggccgacuacagcgugcuguacaacagcgccagcuucagcaccuucaagugcuacggcgugagccccaccaagcugaacgaccugugcuucaccaacguguacgccgacagcuucgugaucagaggcgacgaagugcggcagaucgcccccggacagacaggcaagaucgccgacuacaacuacaagcugcccgacgacuucaccggcugcgugaucgccuggaacagcaacaaccuggacagcaaagucggcggcaacuacaacuaccuguaccggcuguuccggaaguccaaccugaagcccuucgagcgggacaucagcaccgagaucuaccaggccggcagcacccccugcaacggcguggaaggcuucaacugcuacuucccacugcagagcuacggcuuccagcccacauacggcgugggcuaccagcccuacagagugguggugcugagcuucgagcugcugcacgcccccgccacagugugcggccccaagaaaagcaccaaccuggucaagaacaaaugcgugaacuucugagcucgcuuucuugcuguccaauuucuauuaaagguuccuuuguucccuaaguccaacuacuaaacugggggauauuaugaagggccuugagcaucuggauucugccuaauaaaaaacauuuauuuucauugcaaaaaaaaaaaaaaaaaaaaaaaaaaaaaaaaaaaaaaaaaaaaaaaaaaaaaaaaaaaaaaaaaaaaaaaaaaaaaaaaaaaaaaaaaaaaaaaaaaaa

SEQ ID NO: 68 - RNA, 1013 nt, Artificial Sequence
  SARS-CoV-2 variant RBD mRNA (Brazilian variant)
aggagacccaagcuacauuugcuucugacacaacuguguucacuagcaaccucaaacagacaccgccaccauguucguguuccuggugcugcugccccuggugagcagcagagugcagcccaccgagagcaucgugcgguuccccaacaucaccaaccugugccccuucggcgagguguucaacgccaccagauucgccagcguguacgccuggaaccggaagcggaucagcaacugcguggccgacuacagcgugcuguacaacagcgccagcuucagcaccuucaagugcuacggcgugagccccaccaagcugaacgaccugugcuucaccaacguguacgccgacagcuucgugaucagaggcgacgaagugcggcagaucgcccccggacagacaggcacgaucgccgacuacaacuacaagcugcccgacgacuucaccggcugcgugaucgccuggaacagcaacaaccuggacagcaaagucggcggcaacuacaacuaccuguaccggcuguuccggaaguccaaccugaagcccuucgagcgggacaucagcaccgagaucuaccaggccggcagcacccccugcaacggcgugaaaggcuucaacugcuacuucccacugcagagcuacggcuuccagcccacauacggcgugggcuaccagcccuacagagugguggugcugagcuucgagcugcugcacgcccccgccacagugugcggccccaagaaaagcaccaaccuggucaagaacaaaugcgugaacuucugagcucgcuuucuugcuguccaauuucuauuaaagguuccuuuguucccuaaguccaacuacuaaacugggggauauuaugaagggccuugagcaucuggauucugccuaauaaaaaacauuuauuuucauugcaaaaaaaaaaaaaaaaaaaaaaaaaaaaaaaaaaaaaaaaaaaaaaaaaaaaaaaaaaaaaaaaaaaaaaaaaaaaaaaaaaaaaaaaaaaaaaaaaaaa

SEQ ID NO: 69 - RNA, 1013 nt, Artificial Sequence
  SARS-CoV-2 variant RBD mRNA (California variant)
aggagacccaagcuacauuugcuucugacacaacuguguucacuagcaaccucaaacagacaccgccaccauguucguguuccuggugcugcugccccuggugagcagcagagugcagcccaccgagagcaucgugcgguuccccaacaucaccaaccugugccccuucggcgagguguucaacgccaccagauucgccagcguguacgccuggaaccggaagcggaucagcaacugcguggccgacuacagcgugcuguacaacagcgccagcuucagcaccuucaagugcuacggcgugagccccaccaagcugaacgaccugugcuucaccaacguguacgccgacagcuucgugaucagaggcgacgaagugcggcagaucgcccccggacagacaggcaagaucgccgacuacaacuacaagcugcccgacgacuucaccggcugcgugaucgccuggaacagcaacaaccuggacagcaaagucggcggcaacuacaacuaccgguaccggcuguuccggaaguccaaccugaagcccuucgagcgggacaucagcaccgagaucuaccaggccggcagcacccccugcaacggcguggaaggcuucaacugcuacuucccacugcagagcuacggcuuccagcccacaaacggcgugggcuaccagcccuacagagugguggugcugagcuucgagcugcugcacgcccccgccacagugugcggccccaagaaaagcaccaaccuggucaagaacaaaugcgugaacuucugagcucgcuuucuugcuguccaauuucuauuaaagguuccuuuguucccuaaguccaacuacuaaacugggggauauuaugaagggccuugagcaucuggauucugccuaauaaaaaacauuuauuuucauugcaaaaaaaaaaaaaaaaaaaaaaaaaaaaaaaaaaaaaaaaaaaaaaaaaaaaaaaaaaaaaaaaaaaaaaaaaaaaaaaaaaaaaaaaaaaaaaaaaaaa

SEQ ID NO: 70 - RNA, 1013 nt, Artificial Sequence
  SARS-CoV-2 variant RBD mRNA (Indian variant)
aggagacccaagcuacauuugcuucugacacaacuguguucacuagcaaccucaaacagacaccgccaccauguucguguuccuggugcugcugccccuggugagcagcagagugcagcccaccgagagcaucgugcgguuccccaacaucaccaaccugugccccuucggcgagguguucaacgccaccagauucgccagcguguacgccuggaaccggaagcggaucagcaacugcguggccgacuacagcgugcuguacaacagcgccagcuucagcaccuucaagugcuacggcgugagccccaccaagcugaacgaccugugcuucaccaacguguacgccgacagcuucgugaucagaggcgacgaagugcggcagaucgcccccggacagacaggcaagaucgccgacuacaacuacaagcugcccgacgacuucaccggcugcgugaucgccuggaacagcaacaaccuggacagcaaagucggcggcaacuacaacuaccgguaccggcuguuccggaaguccaaccugaagcccuucgagcgggacaucagcaccgagaucuaccaggccggcagcacccccugcaacggcgugcaaggcuucaacugcuacuucccacugcagagcuacggcuuccagcccacaaacggcgugggcuaccagcccuacagagugguggugcugagcuucgagcugcugcacgcccccgccacagugugcggccccaagaaaagcaccaaccuggucaagaacaaaugcgugaacuucugagcucgcuuucuugcuguccaauuucuauuaaagguuccuuuguucccuaaguccaacuacuaaacugggggauauuaugaagggccuugagcaucuggauucugccuaauaaaaaacauuuauuuucauugcaaaaaaaaaaaaaaaaaaaaaaaaaaaaaaaaaaaaaaaaaaaaaaaaaaaaaaaaaaaaaaaaaaaaaaaaaaaaaaaaaaaaaaaaaaaaaaaaaaaa

SEQ ID NO: 71 - RNA, 1013 nt, Artificial Sequence
  SARS-CoV-2 variant RBD mRNA (South African C538S variant)
aggagacccaagcuacauuugcuucugacacaacuguguucacuagcaaccucaaacagacaccgccaccauguucguguuccuggugcugcugccccuggugagcagcagagugcagcccaccgagagcaucgugcgguuccccaacaucaccaaccugugccccuucggcgagguguucaacgccaccagauucgccagcguguacgccuggaaccggaagcggaucagcaacugcguggccgacuacagcgugcuguacaacagcgccagcuucagcaccuucaagugcuacggcgugagccccaccaagcugaacgaccugugcuucaccaacguguacgccgacagcuucgugaucagaggcgacgaagugcggcagaucgcccccggacagacaggcaacaucgccgacuacaacuacaagcugcccgacgacuucaccggcugcgugaucgccuggaacagcaacaaccuggacagcaaagucggcggcaacuacaacuaccuguaccggcuguuccggaaguccaaccugaagcccuucgagcgggacaucagcaccgagaucuaccaggccggcagcacccccugcaacggcgugaaaggcuucaacugcuacuucccacugcagagcuacggcuuccagcccacauacggcgugggcuaccagcccuacagagugguggugcugagcuucgagcugcugcacgcccccgccacagugugcggccccaagaaaagcaccaaccuggucaagaacaaaagcgugaacuucugagcucgcuuucuugcuguccaauuucuauuaaagguuccuuuguucccuaaguccaacuacuaaacugggggauauuaugaagggccuugagcaucuggauucugccuaauaaaaaacauuuauuuucauugcaaaaaaaaaaaaaaaaaaaaaaaaaaaaaaaaaaaaaaaaaaaaaaaaaaaaaaaaaaaaaaaaaaaaaaaaaaaaaaaaaaaaaaaaaaaaaaaaaaaa

SEQ ID NO: 72 - RNA, 1013 nt, Artificial Sequence
  SARS-CoV-2 variant RBD mRNA (UK C538S variant)
aggagacccaagcuacauuugcuucugacacaacuguguucacuagcaaccucaaacagacaccgccaccauguucguguuccuggugcugcugccccuggugagcagcagagugcagcccaccgagagcaucgugcgguuccccaacaucaccaaccugugccccuucggcgagguguucaacgccaccagauucgccagcguguacgccuggaaccggaagcggaucagcaacugcguggccgacuacagcgugcuguacaacagcgccagcuucagcaccuucaagugcuacggcgugagccccaccaagcugaacgaccugugcuucaccaacguguacgccgacagcuucgugaucagaggcgacgaagugcggcagaucgcccccggacagacaggcaagaucgccgacuacaacuacaagcugcccgacgacuucaccggcugcgugaucgccuggaacagcaacaaccuggacagcaaagucggcggcaacuacaacuaccuguaccggcuguuccggaaguccaaccugaagcccuucgagcgggacaucagcaccgagaucuaccaggccggcagcacccccugcaacggcguggaaggcuucaacugcuacuucccacugcagagcuacggcuuccagcccacauacggcgugggcuaccagcccuacagagugguggugcugagcuucgagcugcugcacgcccccgccacagugugcggccccaagaaaagcaccaaccuggucaagaacaaaagcgugaacuucugagcucgcuuucuugcuguccaauuucuauuaaagguuccuuuguucccuaaguccaacuacuaaacugggggauauuaugaagggccuugagcaucuggauucugccuaauaaaaaacauuuauuuucauugcaaaaaaaaaaaaaaaaaaaaaaaaaaaaaaaaaaaaaaaaaaaaaaaaaaaaaaaaaaaaaaaaaaaaaaaaaaaaaaaaaaaaaaaaaaaaaaaaaaaa

SEQ ID NO: 73 - RNA, 1013 nt, Artificial Sequence
  SARS-CoV-2 variant RBD mRNA (Brazilian C538S variant)
aggagacccaagcuacauuugcuucugacacaacuguguucacuagcaaccucaaacagacaccgccaccauguucguguuccuggugcugcugccccuggugagcagcagagugcagcccaccgagagcaucgugcgguuccccaacaucaccaaccugugccccuucggcgagguguucaacgccaccagauucgccagcguguacgccuggaaccggaagcggaucagcaacugcguggccgacuacagcgugcuguacaacagcgccagcuucagcaccuucaagugcuacggcgugagccccaccaagcugaacgaccugugcuucaccaacguguacgccgacagcuucgugaucagaggcgacgaagugcggcagaucgcccccggacagacaggcacgaucgccgacuacaacuacaagcugcccgacgacuucaccggcugcgugaucgccuggaacagcaacaaccuggacagcaaagucggcggcaacuacaacuaccuguaccggcuguuccggaaguccaaccugaagcccuucgagcgggacaucagcaccgagaucuaccaggccggcagcacccccugcaacggcgugaaaggcuucaacugcuacuucccacugcagagcuacggcuuccagcccacauacggcgugggcuaccagcccuacagagugguggugcugagcuucgagcugcugcacgcccccgccacagugugcggccccaagaaaagcaccaaccuggucaagaacaaaagcgugaacuucugagcucgcuuucuugcuguccaauuucuauuaaagguuccuuuguucccuaaguccaacuacuaaacugggggauauuaugaagggccuugagcaucuggauucugccuaauaaaaaacauuuauuuucauugcaaaaaaaaaaaaaaaaaaaaaaaaaaaaaaaaaaaaaaaaaaaaaaaaaaaaaaaaaaaaaaaaaaaaaaaaaaaaaaaaaaaaaaaaaaaaaaaaaaaa

SEQ ID NO: 74 - RNA, 1013 nt, Artificial Sequence
  SARS-CoV-2 variant RBD mRNA (California C538S variant)
aggagacccaagcuacauuugcuucugacacaacuguguucacuagcaaccucaaacagacaccgccaccauguucguguuccuggugcugcugccccuggugagcagcagagugcagcccaccgagagcaucgugcgguuccccaacaucaccaaccugugccccuucggcgagguguucaacgccaccagauucgccagcguguacgccuggaaccggaagcggaucagcaacugcguggccgacuacagcgugcuguacaacagcgccagcuucagcaccuucaagugcuacggcgugagccccaccaagcugaacgaccugugcuucaccaacguguacgccgacagcuucgugaucagaggcgacgaagugcggcagaucgcccccggacagacaggcaagaucgccgacuacaacuacaagcugcccgacgacuucaccggcugcgugaucgccuggaacagcaacaaccuggacagcaaagucggcggcaacuacaacuaccgguaccggcuguuccggaaguccaaccugaagcccuucgagcgggacaucagcaccgagaucuaccaggccggcagcacccccugcaacggcguggaaggcuucaacugcuacuucccacugcagagcuacggcuuccagcccacaaacggcgugggcuaccagcccuacagagugguggugcugagcuucgagcugcugcacgcccccgccacagugugcggccccaagaaaagcaccaaccuggucaagaacaaaagcgugaacuucugagcucgcuuucuugcuguccaauuucuauuaaagguuccuuuguucccuaaguccaacuacuaaacugggggauauuaugaagggccuugagcaucuggauucugccuaauaaaaaacauuuauuuucauugcaaaaaaaaaaaaaaaaaaaaaaaaaaaaaaaaaaaaaaaaaaaaaaaaaaaaaaaaaaaaaaaaaaaaaaaaaaaaaaaaaaaaaaaaaaaaaaaaaaaa

SEQ ID NO: 75 - RNA, 1013 nt, Artificial Sequence
  SARS-CoV-2 variant RBD mRNA (Indian C538S variant)
aggagacccaagcuacauuugcuucugacacaacuguguucacuagcaaccucaaacagacaccgccaccauguucguguuccuggugcugcugccccuggugagcagcagagugcagcccaccgagagcaucgugcgguuccccaacaucaccaaccugugccccuucggcgagguguucaacgccaccagauucgccagcguguacgccuggaaccggaagcggaucagcaacugcguggccgacuacagcgugcuguacaacagcgccagcuucagcaccuucaagugcuacggcgugagccccaccaagcugaacgaccugugcuucaccaacguguacgccgacagcuucgugaucagaggcgacgaagugcggcagaucgcccccggacagacaggcaagaucgccgacuacaacuacaagcugcccgacgacuucaccggcugcgugaucgccuggaacagcaacaaccuggacagcaaagucggcggcaacuacaacuaccgguaccggcuguuccggaaguccaaccugaagcccuucgagcgggacaucagcaccgagaucuaccaggccggcagcacccccugcaacggcgugcaaggcuucaacugcuacuucccacugcagagcuacggcuuccagcccacaaacggcgugggcuaccagcccuacagagugguggugcugagcuucgagcugcugcacgcccccgccacagugugcggccccaagaaaagcaccaaccuggucaagaacaaaagcgugaacuucugagcucgcuuucuugcuguccaauuucuauuaaagguuccuuuguucccuaaguccaacuacuaaacugggggauauuaugaagggccuugagcaucuggauucugccuaauaaaaaacauuuauuuucauugcaaaaaaaaaaaaaaaaaaaaaaaaaaaaaaaaaaaaaaaaaaaaaaaaaaaaaaaaaaaaaaaaaaaaaaaaaaaaaaaaaaaaaaaaaaaaaaaaaaaa

SEQ ID NO: 76 - RNA, 1013 nt, Artificial Sequence
  SARS-CoV-2 variant RBD mRNA (combination variant 1)
aggagacccaagcuacauuugcuucugacacaacuguguucacuagcaaccucaaacagacaccgccaccauguucguguuccuggugcugcugccccuggugagcagcagagugcagcccaccgagagcaucgugcgguuccccaacaucaccaaccugugccccuucggcgagguguucaacgccaccagauucgccagcguguacgccuggaaccggaagcggaucagcaacugcguggccgacuacagcgugcuguacaacagcgccagcuucagcaccuucaagugcuacggcgugagccccaccaagcugaacgaccugugcuucaccaacguguacgccgacagcuucgugaucagaggcgacgaagugcggcagaucgcccccggacagacaggcaagaucgccgacuacaacuacaagcugcccgacgacuucaccggcugcgugaucgccuggaacagcaagaaccuggacagcaaagucggcggcaacuacaacuaccgguaccggcuguuccggaaguccaaccugaagcccuucgagcgggacaucagcaccgagaucuaccaggucggcagcacccccugcaacggcgcggaaggcuucaacugcuacuucccacugcagagcuacggcuuccagcccacaaacggcgugggcuaccagcccuacagagugguggugcugagcuucgagcugcugcacgcccccgccacagugugcggccccaagaaaagcaccaaccuggucaagaacaaaugcgugaacuucugagcucgcuuucuugcuguccaauuucuauuaaagguuccuuuguucccuaaguccaacuacuaaacugggggauauuaugaagggccuugagcaucuggauucugccuaauaaaaaacauuuauuuucauugcaaaaaaaaaaaaaaaaaaaaaaaaaaaaaaaaaaaaaaaaaaaaaaaaaaaaaaaaaaaaaaaaaaaaaaaaaaaaaaaaaaaaaaaaaaaaaaaaaaaa

SEQ ID NO: 77 - RNA, 1013 nt, Artificial Sequence
  SARS-CoV-2 variant RBD mRNA (combination variant 2)
aggagacccaagcuacauuugcuucugacacaacuguguucacuagcaaccucaaacagacaccgccaccauguucguguuccuggugcugcugccccuggugagcagcagagugcagcccaccgagagcaucgugcgguuccccaacaucaccaaccugugccccuucggcgagguguucaacgccaccagauucgccagcguguacgccuggaaccggaagcggaucagcaacugcguggccgacuacagcgugcuguacaacagcgccagcuucagcaccuucaagugcuacggcgugagccccaccaagcugaacgaccugugcuucaccaacguguacgccgacagcuucgugaucagaggcgacgaagugcggcagaucgcccccggacagacaggcaagaucgccgacuacaacuacaagcugcccgacgacuucaccggcugcgugaucgccuggaacagcaacaaccuggacagcaaagucggcggcaacuacaacuaccuguaccggcuguuccggaaguccaaccugaagcccuucgagcgggacaucagcaccgagaucuaccaggccggcagaacccccugcaacggcguggaaggcuucaacugcuaccucccacugcagagcuacggcuuccagcccacaaacggcgugggcuaccagcccuacagagugguggugcugagcuucgagcugcugcacgcccccgccacagugugcggccccaagaaaagcaccaaccuggucaagaacaaaugcgugaacuucugagcucgcuuucuugcuguccaauuucuauuaaagguuccuuuguucccuaaguccaacuacuaaacugggggauauuaugaagggccuugagcaucuggauucugccuaauaaaaaacauuuauuuucauugcaaaaaaaaaaaaaaaaaaaaaaaaaaaaaaaaaaaaaaaaaaaaaaaaaaaaaaaaaaaaaaaaaaaaaaaaaaaaaaaaaaaaaaaaaaaaaaaaaaaa

SEQ ID NO: 78 - RNA, 1013 nt, Artificial Sequence
  SARS-CoV-2 variant RBD mRNA (combination variant 3)
aggagacccaagcuacauuugcuucugacacaacuguguucacuagcaaccucaaacagacaccgccaccauguucguguuccuggugcugcugccccuggugagcagcagagugcagcccaccgagagcaucgugcgguuccccaacaucaccaaccugugccccuucggcgagguguucaacgccaccagauucgccagcguguacgccuggaaccggaagcggaucagcaacugcguggccgacuacagcgugcuguacaacagcgccagcuucagcaccuucaagugcuacggcgugagccccaccaagcugaacgaccugugcuucaccaacguguacgccgacagcuucgugaucagaggcgacgaagugcggcagaucgcccccggacagacaggcaacaucgccgacuacaacuacaagcugcccgacgacuucaccggcugcgugaucgccuggaacagcaacaaccuggacagcaaagucggcggcaacuacaacuaccuguaccggcuguuccggaaguccaaccugaagcccuucgagcgggacaucagcaccgagaucuaccaggccggcagaacccccugcaacggcgugaaaggcuucaacugcuacuucccacugcagagcuacggcuuccagcccacauacggcgugggcuaccagcccuacagagugguggugcugagcuucgagcugcugcacgcccccgccacagugugcggccccaagaaaagcaccaaccuggucaagaacaaaugcgugaacuucugagcucgcuuucuugcuguccaauuucuauuaaagguuccuuuguucccuaaguccaacuacuaaacugggggauauuaugaagggccuugagcaucuggauucugccuaauaaaaaacauuuauuuucauugcaaaaaaaaaaaaaaaaaaaaaaaaaaaaaaaaaaaaaaaaaaaaaaaaaaaaaaaaaaaaaaaaaaaaaaaaaaaaaaaaaaaaaaaaaaaaaaaaaaaa

SEQ ID NO: 79 - RNA, 1013 nt, Artificial Sequence
  SARS-CoV-2 variant RBD mRNA (combination variant 4)
aggagacccaagcuacauuugcuucugacacaacuguguucacuagcaaccucaaacagacaccgccaccauguucguguuccuggugcugcugccccuggugagcagcagagugcagcccaccgagagcaucgugcgguuccccaacaucaccaaccugugccccuucggcgagguguucaacgccaccagauucgccagcguguacgccuggaaccggaagcggaucagcaacugcguggccgacuacagcgugcuguacaacagcgccagcuucagcaccuucaagugcuacggcgugagccccaccaagcugaacgaccugugcuucaccaacguguacgccgacagcuucgugaucagaggcgacgaagugcggcagaucgcccccggacagacaggcaagaucgccgacuacaacuacaagcugcccgacgacuucaccggcugcgugaucgccuggaacagcaacaaccuggacagcaaagucggcggcaacuacaacuaccuguaccggcuguuccggaaguccaaccugaagcccuucgagcgggacaucagcaccgagaucuaccaggccggcagcacccccugcaacggcguggaaggcagcaacugcuaccucccacugcagagcuacggcuuccagcccacaaacggcgugggcuaccagcccuacagagugguggugcugagcuucgagcugcugcacgcccccgccacagugugcggccccaagaaaagcaccaaccuggucaagaacaaaugcgugaacuucugagcucgcuuucuugcuguccaauuucuauuaaagguuccuuuguucccuaaguccaacuacuaaacugggggauauuaugaagggccuugagcaucuggauucugccuaauaaaaaacauuuauuuucauugcaaaaaaaaaaaaaaaaaaaaaaaaaaaaaaaaaaaaaaaaaaaaaaaaaaaaaaaaaaaaaaaaaaaaaaaaaaaaaaaaaaaaaaaaaaaaaaaaaaaa

SEQ ID NO: 80 - protein, 236 aa, Artificial Sequence
  spike protein signal sequence added SARS-CoV-2 variant RBD (South African variant)
MFVFLVLLPLVSSRVQPTESIVRFPNITNLCPFGEVFNATRFASVYAWNRKRISNCVADYSVLYNSASFSTFKCYGVSPTKLNDLCFTNVYADSFVIRGDEVRQIAPGQTGNIADYNYKLPDDFTGCVIAWNSNNLDSKVGGNYNYLYRLFRKSNLKPFERDISTEIYQAGSTPCNGVKGFNCYFPLQSYGFQPTYGVGYQPYRVVVLSFELLHAPATVCGPKKSTNLVKNKCVNF

SEQ ID NO: 81 - protein, 236 aa, Artificial Sequence
  spike protein signal sequence added SARS-CoV-2 variant RBD (UK variant)
MFVFLVLLPLVSSRVQPTESIVRFPNITNLCPFGEVFNATRFASVYAWNRKRISNCVADYSVLYNSASFSTFKCYGVSPTKLNDLCFTNVYADSFVIRGDEVRQIAPGQTGKIADYNYKLPDDFTGCVIAWNSNNLDSKVGGNYNYLYRLFRKSNLKPFERDISTEIYQAGSTPCNGVEGFNCYFPLQSYGFQPTYGVGYQPYRVVVLSFELLHAPATVCGPKKSTNLVKNKCVNF

SEQ ID NO: 82 - protein, 236 aa, Artificial Sequence
  spike protein signal sequence added SARS-CoV-2 variant RBD (Brazilian variant)
MFVFLVLLPLVSSRVQPTESIVRFPNITNLCPFGEVFNATRFASVYAWNRKRISNCVADYSVLYNSASFSTFKCYGVSPTKLNDLCFTNVYADSFVIRGDEVRQIAPGQTGTIADYNYKLPDDFTGCVIAWNSNNLDSKVGGNYNYLYRLFRKSNLKPFERDISTEIYQAGSTPCNGVKGFNCYFPLQSYGFQPTYGVGYQPYRVVVLSFELLHAPATVCGPKKSTNLVKNKCVNF

SEQ ID NO: 83 - protein, 236 aa, Artificial Sequence
  spike protein signal sequence added SARS-CoV-2 variant RBD (California variant)
MFVFLVLLPLVSSRVQPTESIVRFPNITNLCPFGEVFNATRFASVYAWNRKRISNCVADYSVLYNSASFSTFKCYGVSPTKLNDLCFTNVYADSFVIRGDEVRQIAPGQTGKIADYNYKLPDDFTGCVIAWNSNNLDSKVGGNYNYRYRLFRKSNLKPFERDISTEIYQAGSTPCNGVEGFNCYFPLQSYGFQPTNGVGYQPYRVVVLSFELLHAPATVCGPKKSTNLVKNKCVNF

SEQ ID NO: 84 - protein, 236 aa, Artificial Sequence
  spike protein signal sequence added SARS-CoV-2 variant RBD (Indian variant)
MFVFLVLLPLVSSRVQPTESIVRFPNITNLCPFGEVFNATRFASVYAWNRKRISNCVADYSVLYNSASFSTFKCYGVSPTKLNDLCFTNVYADSFVIRGDEVRQIAPGQTGKIADYNYKLPDDFTGCVIAWNSNNLDSKVGGNYNYRYRLFRKSNLKPFERDISTEIYQAGSTPCNGVQGFNCYFPLQSYGFQPTNGVGYQPYRVVVLSFELLHAPATVCGPKKSTNLVKNKCVNF

SEQ ID NO: 85 - protein, 236 aa, Artificial Sequence
  spike protein signal sequence added SARS-CoV-2 variant RBD (South African C538S variant)
MFVFLVLLPLVSSRVQPTESIVRFPNITNLCPFGEVFNATRFASVYAWNRKRISNCVADYSVLYNSASFSTFKCYGVSPTKLNDLCFTNVYADSFVIRGDEVRQIAPGQTGNIADYNYKLPDDFTGCVIAWNSNNLDSKVGGNYNYLYRLFRKSNLKPFERDISTEIYQAGSTPCNGVKGFNCYFPLQSYGFQPTYGVGYQPYRVVVLSFELLHAPATVCGPKKSTNLVKNKSVNF

SEQ ID NO: 86 - protein, 236 aa, Artificial Sequence
  spike protein signal sequence added SARS-CoV-2 variant RBD (UK C538S variant)
MFVFLVLLPLVSSRVQPTESIVRFPNITNLCPFGEVFNATRFASVYAWNRKRISNCVADYSVLYNSASFSTFKCYGVSPTKLNDLCFTNVYADSFVIRGDEVRQIAPGQTGKIADYNYKLPDDFTGCVIAWNSNNLDSKVGGNYNYLYRLFRKSNLKPFERDISTEIYQAGSTPCNGVEGFNCYFPLQSYGFQPTYGVGYQPYRVVVLSFELLHAPATVCGPKKSTNLVKNKSVNF

SEQ ID NO: 87 - protein, 236 aa, Artificial Sequence
  spike protein signal sequence added SARS-CoV-2 variant RBD (Brazilian C538S variant)
MFVFLVLLPLVSSRVQPTESIVRFPNITNLCPFGEVFNATRFASVYAWNRKRISNCVADYSVLYNSASFSTFKCYGVSPTKLNDLCFTNVYADSFVIRGDEVRQIAPGQTGTIADYNYKLPDDFTGCVIAWNSNNLDSKVGGNYNYLYRLFRKSNLKPFERDISTEIYQAGSTPCNGVKGFNCYFPLQSYGFQPTYGVGYQPYRVVVLSFELLHAPATVCGPKKSTNLVKNKSVNF

SEQ ID NO: 88 - protein, 236 aa, Artificial Sequence
  spike protein signal sequence added SARS-CoV-2 variant RBD (California C538S variant)
MFVFLVLLPLVSSRVQPTESIVRFPNITNLCPFGEVFNATRFASVYAWNRKRISNCVADYSVLYNSASFSTFKCYGVSPTKLNDLCFTNVYADSFVIRGDEVRQIAPGQTGKIADYNYKLPDDFTGCVIAWNSNNLDSKVGGNYNYRYRLFRKSNLKPFERDISTEIYQAGSTPCNGVEGFNCYFPLQSYGFQPTNGVGYQPYRVVVLSFELLHAPATVCGPKKSTNLVKNKSVNF

SEQ ID NO: 89 - protein, 236 aa, Artificial Sequence
  spike protein signal sequence added SARS-CoV-2 variant RBD (Indian C538S variant)
MFVFLVLLPLVSSRVQPTESIVRFPNITNLCPFGEVFNATRFASVYAWNRKRISNCVADYSVLYNSASFSTFKCYGVSPTKLNDLCFTNVYADSFVIRGDEVRQIAPGQTGKIADYNYKLPDDFTGCVIAWNSNNLDSKVGGNYNYRYRLFRKSNLKPFERDISTEIYQAGSTPCNGVQGFNCYFPLQSYGFQPTNGVGYQPYRVVVLSFELLHAPATVCGPKKSTNLVKNKSVNF

SEQ ID NO: 90 - protein, 236 aa, Artificial Sequence
  spike protein signal sequence added SARS-CoV-2 variant RBD (combination variant 1)
MFVFLVLLPLVSSRVQPTESIVRFPNITNLCPFGEVFNATRFASVYAWNRKRISNCVADYSVLYNSASFSTFKCYGVSPTKLNDLCFTNVYADSFVIRGDEVRQIAPGQTGKIADYNYKLPDDFTGCVIAWNSKNLDSKVGGNYNYRYRLFRKSNLKPFERDISTEIYQVGSTPCNGAEGFNCYFPLQSYGFQPTNGVGYQPYRVVVLSFELLHAPATVCGPKKSTNLVKNKCVNF

SEQ ID NO: 91 - protein, 236 aa, Artificial Sequence
  spike protein signal sequence added SARS-CoV-2 variant RBD (combination variant 2)
MFVFLVLLPLVSSRVQPTESIVRFPNITNLCPFGEVFNATRFASVYAWNRKRISNCVADYSVLYNSASFSTFKCYGVSPTKLNDLCFTNVYADSFVIRGDEVRQIAPGQTGKIADYNYKLPDDFTGCVIAWNSNNLDSKVGGNYNYLYRLFRKSNLKPFERDISTEIYQAGRTPCNGVEGFNCYLPLQSYGFQPTNGVGYQPYRVVVLSFELLHAPATVCGPKKSTNLVKNKCVNF

SEQ ID NO: 92 - protein, 236 aa, Artificial Sequence
  spike protein signal sequence added SARS-CoV-2 variant RBD (combination variant 3)
MFVFLVLLPLVSSRVQPTESIVRFPNITNLCPFGEVFNATRFASVYAWNRKRISNCVADYSVLYNSASFSTFKCYGVSPTKLNDLCFTNVYADSFVIRGDEVRQIAPGQTGNIADYNYKLPDDFTGCVIAWNSNNLDSKVGGNYNYLYRLFRKSNLKPFERDISTEIYQAGRTPCNGVKGFNCYFPLQSYGFQPTYGVGYQPYRVVVLSFELLHAPATVCGPKKSTNLVKNKCVNF

SEQ ID NO: 93 - protein, 236 aa, Artificial Sequence
  spike protein signal sequence added SARS-CoV-2 variant RBD (combination variant 4)
MFVFLVLLPLVSSRVQPTESIVRFPNITNLCPFGEVFNATRFASVYAWNRKRISNCVADYSVLYNSASFSTFKCYGVSPTKLNDLCFTNVYADSFVIRGDEVRQIAPGQTGKIADYNYKLPDDFTGCVIAWNSNNLDSKVGGNYNYLYRLFRKSNLKPFERDISTEIYQAGSTPCNGVEGSNCYLPLQSYGFQPTNGVGYQPYRVVVLSFELLHAPATVCGPKKSTNLVKNKCVNF

SEQ ID NO: 94 - protein, 223 aa, Artificial Sequence
  SARS-CoV-2 variant RBD (South African variant)
RVQPTESIVRFPNITNLCPFGEVFNATRFASVYAWNRKRISNCVADYSVLYNSASFSTFKCYGVSPTKLNDLCFTNVYADSFVIRGDEVRQIAPGQTGNIADYNYKLPDDFTGCVIAWNSNNLDSKVGGNYNYLYRLFRKSNLKPFERDISTEIYQAGSTPCNGVKGFNCYFPLQSYGFQPTYGVGYQPYRVVVLSFELLHAPATVCGPKKSTNLVKNKCVNF

SEQ ID NO: 95 - protein, 223 aa, Artificial Sequence
  SARS-CoV-2 variant RBD (UK variant)
RVQPTESIVRFPNITNLCPFGEVFNATRFASVYAWNRKRISNCVADYSVLYNSASFSTFKCYGVSPTKLNDLCFTNVYADSFVIRGDEVRQIAPGQTGKIADYNYKLPDDFTGCVIAWNSNNLDSKVGGNYNYLYRLFRKSNLKPFERDISTEIYQAGSTPCNGVEGFNCYFPLQSYGFQPTYGVGYQPYRVVVLSFELLHAPATVCGPKKSTNLVKNKCVNF

SEQ ID NO: 96 - protein, 223 aa, Artificial Sequence
  SARS-CoV-2 variant RBD (Brazilian variant)
RVQPTESIVRFPNITNLCPFGEVFNATRFASVYAWNRKRISNCVADYSVLYNSASFSTFKCYGVSPTKLNDLCFTNVYADSFVIRGDEVRQIAPGQTGTIADYNYKLPDDFTGCVIAWNSNNLDSKVGGNYNYLYRLFRKSNLKPFERDISTEIYQAGSTPCNGVKGFNCYFPLQSYGFQPTYGVGYQPYRVVVLSFELLHAPATVCGPKKSTNLVKNKCVNF

SEQ ID NO: 97 - protein, 223 aa, Artificial Sequence
  SARS-CoV-2 variant RBD (California variant)
RVQPTESIVRFPNITNLCPFGEVFNATRFASVYAWNRKRISNCVADYSVLYNSASFSTFKCYGVSPTKLNDLCFTNVYADSFVIRGDEVRQIAPGQTGKIADYNYKLPDDFTGCVIAWNSNNLDSKVGGNYNYRYRLFRKSNLKPFERDISTEIYQAGSTPCNGVEGFNCYFPLQSYGFQPTNGVGYQPYRVVVLSFELLHAPATVCGPKKSTNLVKNKCVNF

SEQ ID NO: 98 - protein, 223 aa, Artificial Sequence
  SARS-CoV-2 variant RBD (Indian variant)
RVQPTESIVRFPNITNLCPFGEVFNATRFASVYAWNRKRISNCVADYSVLYNSASFSTFKCYGVSPTKLNDLCFTNVYADSFVIRGDEVRQIAPGQTGKIADYNYKLPDDFTGCVIAWNSNNLDSKVGGNYNYRYRLFRKSNLKPFERDISTEIYQAGSTPCNGVQGFNCYFPLQSYGFQPTNGVGYQPYRVVVLSFELLHAPATVCGPKKSTNLVKNKCVNF

SEQ ID NO: 99 - protein, 223 aa, Artificial Sequence
  SARS-CoV-2 variant RBD (South African C538S variant)
RVQPTESIVRFPNITNLCPFGEVFNATRFASVYAWNRKRISNCVADYSVLYNSASFSTFKCYGVSPTKLNDLCFTNVYADSFVIRGDEVRQIAPGQTGNIADYNYKLPDDFTGCVIAWNSNNLDSKVGGNYNYLYRLFRKSNLKPFERDISTEIYQAGSTPCNGVKGFNCYFPLQSYGFQPTYGVGYQPYRVVVLSFELLHAPATVCGPKKSTNLVKNKSVNF

SEQ ID NO: 100 - protein, 223 aa, Artificial Sequence
  SARS-CoV-2 variant RBD (UK C538S variant)
RVQPTESIVRFPNITNLCPFGEVFNATRFASVYAWNRKRISNCVADYSVLYNSASFSTFKCYGVSPTKLNDLCFTNVYADSFVIRGDEVRQIAPGQTGKIADYNYKLPDDFTGCVIAWNSNNLDSKVGGNYNYLYRLFRKSNLKPFERDISTEIYQAGSTPCNGVEGFNCYFPLQSYGFQPTYGVGYQPYRVVVLSFELLHAPATVCGPKKSTNLVKNKSVNF

SEQ ID NO: 101 - protein, 223 aa, Artificial Sequence
  SARS-CoV-2 variant RBD (Brazilian C538S variant)
RVQPTESIVRFPNITNLCPFGEVFNATRFASVYAWNRKRISNCVADYSVLYNSASFSTFKCYGVSPTKLNDLCFTNVYADSFVIRGDEVRQIAPGQTGTIADYNYKLPDDFTGCVIAWNSNNLDSKVGGNYNYLYRLFRKSNLKPFERDISTEIYQAGSTPCNGVKGFNCYFPLQSYGFQPTYGVGYQPYRVVVLSFELLHAPATVCGPKKSTNLVKNKSVNF

SEQ ID NO: 102 - protein, 223 aa, Artificial Sequence
  SARS-CoV-2 variant RBD (California C538S variant)
RVQPTESIVRFPNITNLCPFGEVFNATRFASVYAWNRKRISNCVADYSVLYNSASFSTFKCYGVSPTKLNDLCFTNVYADSFVIRGDEVRQIAPGQTGKIADYNYKLPDDFTGCVIAWNSNNLDSKVGGNYNYRYRLFRKSNLKPFERDISTEIYQAGSTPCNGVEGFNCYFPLQSYGFQPTNGVGYQPYRVVVLSFELLHAPATVCGPKKSTNLVKNKSVNF

SEQ ID NO: 103 - protein, 223 aa, Artificial Sequence
  SARS-CoV-2 variant RBD (Indian C538S variant)
RVQPTESIVRFPNITNLCPFGEVFNATRFASVYAWNRKRISNCVADYSVLYNSASFSTFKCYGVSPTKLNDLCFTNVYADSFVIRGDEVRQIAPGQTGKIADYNYKLPDDFTGCVIAWNSNNLDSKVGGNYNYRYRLFRKSNLKPFERDISTEIYQAGSTPCNGVQGFNCYFPLQSYGFQPTNGVGYQPYRVVVLSFELLHAPATVCGPKKSTNLVKNKSVNF

SEQ ID NO: 104 - protein, 223 aa, Artificial Sequence
  SARS-CoV-2 variant RBD (Combination  variant 1)
RVQPTESIVRFPNITNLCPFGEVFNATRFASVYAWNRKRISNCVADYSVLYNSASFSTFKCYGVSPTKLNDLCFTNVYADSFVIRGDEVRQIAPGQTGKIADYNYKLPDDFTGCVIAWNSKNLDSKVGGNYNYRYRLFRKSNLKPFERDISTEIYQVGSTPCNGAEGFNCYFPLQSYGFQPTNGVGYQPYRVVVLSFELLHAPATVCGPKKSTNLVKNKCVNF

SEQ ID NO: 105 - protein, 223 aa, Artificial Sequence
  SARS-CoV-2 variant RBD (Combination  variant 2)
RVQPTESIVRFPNITNLCPFGEVFNATRFASVYAWNRKRISNCVADYSVLYNSASFSTFKCYGVSPTKLNDLCFTNVYADSFVIRGDEVRQIAPGQTGKIADYNYKLPDDFTGCVIAWNSNNLDSKVGGNYNYLYRLFRKSNLKPFERDISTEIYQAGRTPCNGVEGFNCYLPLQSYGFQPTNGVGYQPYRVVVLSFELLHAPATVCGPKKSTNLVKNKCVNF

SEQ ID NO: 106 - protein, 223 aa, Artificial Sequence
  SARS-CoV-2 variant RBD (Combination  variant 3)
RVQPTESIVRFPNITNLCPFGEVFNATRFASVYAWNRKRISNCVADYSVLYNSASFSTFKCYGVSPTKLNDLCFTNVYADSFVIRGDEVRQIAPGQTGNIADYNYKLPDDFTGCVIAWNSNNLDSKVGGNYNYLYRLFRKSNLKPFERDISTEIYQAGRTPCNGVKGFNCYFPLQSYGFQPTYGVGYQPYRVVVLSFELLHAPATVCGPKKSTNLVKNKCVNF

SEQ ID NO: 107 - protein, 223 aa, Artificial Sequence
  SARS-CoV-2 variant RBD (Combination  variant 4)
RVQPTESIVRFPNITNLCPFGEVFNATRFASVYAWNRKRISNCVADYSVLYNSASFSTFKCYGVSPTKLNDLCFTNVYADSFVIRGDEVRQIAPGQTGKIADYNYKLPDDFTGCVIAWNSNNLDSKVGGNYNYLYRLFRKSNLKPFERDISTEIYQAGSTPCNGVEGSNCYLPLQSYGFQPTNGVGYQPYRVVVLSFELLHAPATVCGPKKSTNLVKNKCVNF